European Patent Application EP 4 316 528 A1, published February 7, 2024. Title: Novel conjugate of immune stimulating IL-2 analog and a preparation method thereof. Applicant: HANMI PHARM. CO., LTD. The sequence listing filed with the application follows.

SEQUENCE LISTING (439 sequences)

SEQ ID NO: 1 - protein, 133 aa, homo sapiens [sequence omitted]

SEQ ID NO: 2 - protein, 132 aa, Artificial Sequence
  IL-2 analog 1
PTSSSTKKTQLQLEHLLLDLQMILNGINNYKNPKLTRMLTFKFYMPKKATELKHLQCLEEELKPLEEVLNLAQSKNFHLRPRDLISNINVIVLELKGSETTFMCEYADETATIVEFLNRWITFSQSIISTLT

SEQ ID NO: 3 - protein, 132 aa, Artificial Sequence
  IL-2 analog 2
PTSSSTKKTQLQLEHLLLDLQMILNGINNYKNPKLTRMLTFKFYMPKKATELKHLQCLEEELKPLEEVLNLAQSKNFHLRPRDLICNINVIVLELKGSETTFMCEYADETATIVEFLNRWITFSQSIISTLT

SEQ ID NO: 4 - protein, 132 aa, Artificial Sequence
  IL-2 analog 3
PTSSSTKKTQLQLEHLLLDLQMILNGINNYCNPKLTRMLTFKFYMPKKATELKHLQCLEEELKPLEEVLNLAQSKNFHLRPRDLISNINVIVLELKGSETTFMCEYADETATIVEFLNRWITFSQSIISTLT

SEQ ID NO: 5 - protein, 132 aa, Artificial Sequence
  IL-2 analog 4
PTSSSTKKTQLQLEHLLLDLQMILNGINNYKNPCLTRMLTFKFYMPKKATELKHLQCLEEELKPLEEVLNLAQSKNFHLRPRDLISNINVIVLELKGSETTFMCEYADETATIVEFLNRWITFSQSIISTLT

SEQ ID NO: 6 - protein, 132 aa, Artificial Sequence
  IL-2 analog 5
PTSSSTKKTQLQLEHLLLDLQMILNGINNYKNPKLTRMLTFCFYMPKKATELKHLQCLEEELKPLEEVLNLAQSKNFHLRPRDLISNINVIVLELKGSETTFMCEYADETATIVEFLNRWITFSQSIISTLT

SEQ ID NO: 7 - protein, 132 aa, Artificial Sequence
  IL-2 analog 6
PTSSSTKKTQLQLEHLLLDLQMILNGINNYKNPKLTRMLTFKFYMPCKATELKHLQCLEEELKPLEEVLNLAQSKNFHLRPRDLISNINVIVLELKGSETTFMCEYADETATIVEFLNRWITFSQSIISTLT

SEQ ID NO: 8 - protein, 132 aa, Artificial Sequence
  IL-2 analog 7
PTSSSTKKTQLQLEHLLLDLQMILNGINNYKNPKLTRMLTFKFYMPKCATELKHLQCLEEELKPLEEVLNLAQSKNFHLRPRDLISNINVIVLELKGSETTFMCEYADETATIVEFLNRWITFSQSIISTLT

SEQ ID NO: 9 - protein, 132 aa, Artificial Sequence
  IL-2 analog 9
PTSSSTKKTQLQLEHLLLDLQMILNGINNYKNPKLTRMLTFKFYMPKKATELKHLQCLEEELKPLEEVLNLAQSCNFHLRPRDLISNINVIVLELKGSETTFMCEYADETATIVEFLNRWITFSQSIISTLT

SEQ ID NO: 10 - protein, 132 aa, Artificial Sequence
  IL-2 analog 10
PTSSSTKKTQLQLEHLLLDLQMILNGINNYKNPKLTAMLTFKFYMPKKATELKHLQCLEEELKPLEEVLNLAQSKNFHLRPRDLISNINVIVLELKGSETTFMCEYADETATIVEFLNRWITFSQSIISTLT

SEQ ID NO: 11 - protein, 132 aa, Artificial Sequence
  IL-2 analog 10
PTSSSTKKTQLQLEHLLLDLQMILNGINNYKNPKLTRMLTKKFYMPKKATELKHLQCLEEELKPLEEVLNLAQSKNFHLRPRDLISNINVIVLELKGSETTFMCEYADETATIVEFLNRWITFSQSIISTLT

SEQ ID NO: 12 - protein, 132 aa, Artificial Sequence
  IL-2 analog 11
PTSSSTKKTQLQLEHLLLDLQMILNGINNYKNPKLTRMLTAKFYMPKKATELKHLQCLEEELKPLEEVLNLAQSKNFHLRPRDLISNINVIVLELKGSETTFMCEYADETATIVEFLNRWITFSQSIISTLT

SEQ ID NO: 13 - protein, 132 aa, Artificial Sequence
  IL-2 analog 12
PTSSSTKKTQLQLEHLLLDLQMILNGINNYKNPKLTAMLTKKFYMPKKATELKHLQCLEEELKPLEEVLNLAQSKNFHLRPRDLISNINVIVLELKGSETTFMCEYADETATIVEFLNRWITFSQSIISTLT

SEQ ID NO: 14 - protein, 132 aa, Artificial Sequence
  IL-2 analog 13
PTSSSTKKTQLQLEHLLLDLQMILNGINNYKNPKLTAMLTAKFYMPKKATELKHLQCLEEELKPLEEVLNLAQSKNFHLRPRDLISNINVIVLELKGSETTFMCEYADETATIVEFLNRWITFSQSIISTLT

SEQ ID NO: 15 - protein, 132 aa, Artificial Sequence
  IL-2 analog 14
PTSSSTKKTQLQLEHLLYDLQMILNGINNYKNPKLTAMLTKKFYMPKKATELKHLQCLEEELKPLEEVLNLAQSKNFHLRPRDLISNINVIVLELKGSETTFMCEYADETATIVEFLNRWITFSQSIISTLT

SEQ ID NO: 16 - protein, 132 aa, Artificial Sequence
  IL-2 analog 15
PTSSSTKKTQLQLEHLLLDLQMILNGINNYKNPKLTAMLTKKFYMPKKATELKHLQCLEEELKPLEEVLNLAQSKNFHLRPRELISNINVIVLELKGSETTFMCEYADETATIVEFLNRWITFSQSIISTLT

SEQ ID NO: 17 - protein, 132 aa, Artificial Sequence
  IL-2 analog 16
PTSSSTKKTQLQLEHLLLDLQMILNGINNYKNPKLTAMLTKKFYMPKKATELKHLQCLEEELKPLEEVLNLAQSKNFHLRPRDLISQINVIVLELKGSETTFMCEYADETATIVEFLNRWITFSQSIISTLT

SEQ ID NO: 18 - protein, 132 aa, Artificial Sequence
  IL-2 analog 17
PTSSSTKKTQLQLEHLLLDLQMILNGINNYKNPKLTAMLTKKFYMPKKATELKHLQCLEEELKPLEEVLNLAQSKNFHLRPRDLISNINTIVLELKGSETTFMCEYADETATIVEFLNRWITFSQSIISTLT

SEQ ID NO: 19 - protein, 132 aa, Artificial Sequence
  IL-2 analog 18
PTSSSTKKTQLQLEHLLLDLQMILNGINNYKNPKLTAMLTKKFYMPKKATELKHLQCLEQELKPLEEVLNLAQSKNFHLRPRDLISNINVIVLELKGSETTFMCEYADETATIVEFLNRWITFSQSIISTLT

SEQ ID NO: 20 - protein, 132 aa, Artificial Sequence
  IL-2 analog 19
PTSSSTKKTQLQLEHLLLDLQMILNGINNYKNPKLTAMLTKKFYMPKKATELKHLQCLEEELKPLEEVLNLAQSKNFHLDPRDLISNINVFVLELKGSETTFMCEYADETATIVEFLNRWITFSQSIISTLT

SEQ ID NO: 21 - protein, 132 aa, Artificial Sequence
  IL-2 analog 20
PTSSSTKKTQLQLEHLLLDLQMILNGINNYKNPKLTAMLTKKFYMPKKATELKHLQCLEEELKPLEEVLNLAQSKNFHLRPRDVVSNINVFVLELKGSETTFMCEYADETATIVEFLNRWITFSQSIISTLT

SEQ ID NO: 22 - protein, 132 aa, Artificial Sequence
  IL-2 analog 21
PTSSSTKKTQLQLEHLLLDLQMILNGINNYKNPKLTAMLTKKFYMPKKATELKHLQCLEEELKPLEEVLNLAQSKNFHFDPRDVVSNINVFVLELKGSETTFMCEYADETATIVEFLNRWITFSQSIISTLT

SEQ ID NO: 23 - protein, 132 aa, Artificial Sequence
  IL-2 analog 22
PTSSSTKKTQVQLEHLLLDLQMILNGINNYKNPKLTAMLTKKFYMPKKATELKHLQCLEEELKPLEEVLNLAQSKNFHLRPRDLISNINVIVLELKGSETTFMCEYADETATIVEFLNRWITFSQSIISTLT

SEQ ID NO: 24 - protein, 132 aa, Artificial Sequence
  IL-2 analog 23
PTSSSTKKTQFQLEHLLLDLQMILNGINNYKNPKLTAMLTKKFYMPKKATELKHLQCLEEELKPLEEVLNLAQSKNFHLRPRDLISNINVIVLELKGSETTFMCEYADETATIVEFLNRWITFSQSIISTLT

SEQ ID NO: 25 - protein, 132 aa, Artificial Sequence
  IL-2 analog 24
PTSSSTKKTQLQLEHLLVDLQMILNGINNYKNPKLTAMLTKKFYMPKKATELKHLQCLEEELKPLEEVLNLAQSKNFHLRPRDLISNINVIVLELKGSETTFMCEYADETATIVEFLNRWITFSQSIISTLT

SEQ ID NO: 26 - protein, 132 aa, Artificial Sequence
  IL-2 analog 25
PTSSSTKKTQLQLEHLLFDLQMILNGINNYKNPKLTAMLTKKFYMPKKATELKHLQCLEEELKPLEEVLNLAQSKNFHLRPRDLISNINVIVLELKGSETTFMCEYADETATIVEFLNRWITFSQSIISTLT

SEQ ID NO: 27 - protein, 132 aa, Artificial Sequence
  IL-2 analog 26
PTSSSTKKTQLQLEHLLLDLQMILNGINNYKNPKLTAMLTKKFYMPKKATELKHLQCLEEELKPLEEVLNLAQSKNFHLRPRDLISNFNVIVLELKGSETTFMCEYADETATIVEFLNRWITFSQSIISTLT

SEQ ID NO: 28 - protein, 132 aa, Artificial Sequence
  IL-2 analog 27
PTSSSTKKTQLQLEHLLLDLQMILNGINNYKNPKLTAMLTKKFYMPKKATELKHLQCLEEELKPLEEVLNLAQSKNFHLRPRDLISNINFIVLELKGSETTFMCEYADETATIVEFLNRWITFSQSIISTLT

SEQ ID NO: 29 - protein, 132 aa, Artificial Sequence
  IL-2 analog 28
PTSSSTKKTQLQLEHLLLDLQMILNGINNYKNPKLTAMLTKKFYMPKKATELKHLQCLEEELKPLEEVLNLAQSKNFHLRPRDLISNINVIVVELKGSETTFMCEYADETATIVEFLNRWITFSQSIISTLT

SEQ ID NO: 30 - protein, 132 aa, Artificial Sequence
  IL-2 analog 29
PTSSSTKKTQLQLEHLLLDLQMILNGINNYKNPKLTAMLTKKFYMPKKATELKHLQCLEEELKPLEEVLNLAQSKNFHLRPRDLISNINVIVLELKGSETTFMCEYADETATIVEFLNRWITFSTSIISTLT

SEQ ID NO: 31 - protein, 132 aa, Artificial Sequence
  IL-2 analog 30
PTSSSTKKTQLQLEHLLLDLQMILNGINNYKNPKLTAMLTFKFYMPKKATELKHLQCLEEELKPLEEVLNLAQSKNFHLDPRDLISNINVFVLELKGSETTFMCEYADETATIVEFLNRWITFSQSIISTLT

SEQ ID NO: 32 - protein, 132 aa, Artificial Sequence
  IL-2 analog 31
PTSSSTKKTQLQLEHLLLDLQMILNGINNYKNPKLTAMLTFKFYMPKKATELKHLQCLEEELKPLEEVLNLAQSKNFHLRPRELISNINVIVLELKGSETTFMCEYADETATIVEFLNRWITFSQSIISTLT

SEQ ID NO: 33 - protein, 132 aa, Artificial Sequence
  IL-2 analog 32
PTSSSTKKTQLQLEHLLLDLQMILNGINNYKNPKLTAMLTFKFYMPKKATELKHLQCLEEELKPLEEVLNLAQSKNFHLDPRELISNINVFVLELKGSETTFMCEYADETATIVEFLNRWITFSQSIISTLT

SEQ ID NO: 34 - protein, 132 aa, Artificial Sequence
  IL-2 analog 33
PTSSSTKKTQLQLEHLLLDLQMILNGINNYKNPKLTAMLTFKFYMPKKATELKHLQCLEEELKPLEEVLNLAQSKNFHFRPRDLISNINVIVLELKGSETTFMCEYADETATIVEFLNRWITFSQSIISTLT

SEQ ID NO: 35 - protein, 132 aa, Artificial Sequence
  IL-2 analog 34
PTSSSTKKTQLQLEHLLLDLQMILNGINNYKNPKLTAMLTFKFYMPKKATELKHLQCLEEELKPLEEVLNLAQSKNFHFRPRELISNINVIVLELKGSETTFMCEYADETATIVEFLNRWITFSQSIISTLT

SEQ ID NO: 36 - protein, 132 aa, Artificial Sequence
  IL-2 analog 35
PTSSSTKKTQLQLEHLLLDLQMILNGINNYKNPKLTAMLTFKFYMPKKATELKHLQCLEEELKPLEEVLNLAQSKNFHLRPRDLISNINVIVFEFKGSETTFMCEYADETATIVEFLNRWITFSQSIISTLT

SEQ ID NO: 37 - protein, 132 aa, Artificial Sequence
  IL-2 analog 36
PTSSSTKKTQLQLEHLLLDLQMILNGINNYKNPKLTAMLTFKFYMPKKATELKHLQCLEEELKPLEEVLNLAQSKNFHLRPRDLISNINVIVFEVKGSETTFMCEYADETATIVEFLNRWITFSQSIISTLT

SEQ ID NO: 38 - protein, 132 aa, Artificial Sequence
  IL-2 analog 37
PTSSSTKKTQLQLEHLLLDLQMILNGINNYKNPKLTAMLTFKFYMPKKATELKHLQCLEEELKPLEEVLNLAQSKNFHLRPRDLISNINVIVFEIKGSETTFMCEYADETATIVEFLNRWITFSQSIISTLT

SEQ ID NO: 39 - protein, 132 aa, Artificial Sequence
  IL-2 analog 38
PTSSSTKKTQLQLEHLLLDLQMILNGINNYKNPKLTAMLTFKFYMPKKATELKHLQCLEEELKPLEEVLNLAQSKNFHLDPRDLISNINVFVFEFKGSETTFMCEYADETATIVEFLNRWITFSQSIISTLT

SEQ ID NO: 40 - protein, 132 aa, Artificial Sequence
  IL-2 analog 39
PTSSSTKKTQLQLEHLLLDLQMILNGINNYKNPKLTAMLTFKFYMPKKATELKHLQCLEEELKPLEEVLNLAQSKNFHLDPRDLISNINVFVFEVKGSETTFMCEYADETATIVEFLNRWITFSQSIISTLT

SEQ ID NO: 41 - protein, 132 aa, Artificial Sequence
  IL-2 analog 40
PTSSSTKKTQLQLEHLLLDLQMILNGINNYKNPKLTAMLTKKFYMPKKATELKHLQCLEEELKPLEEVLNLAQSKNFHLDPRDLISNINVFVFEIKGSETTFMCEYADETATIVEFLNRWITFSQSIISTLT

SEQ ID NO: 42 - protein, 132 aa, Artificial Sequence
  IL-2 analog 41
PTSSSTKKTQLQLEHLLLDLQMILNGINNYKNPKLTRMLTFKFYMPKKATELKHLQCLEEELKPLEEVLNLAQSKNFHFDPRDVVSNINVFVLELKGSETTFMCEYADETATIVEFLNRWITFSQSIISTLT

SEQ ID NO: 43 - protein, 132 aa, Artificial Sequence
  IL-2 analog 42
PTSSSTKKTQLQLEHLLLDLQMILNGINNYKNPKLTAMLTKKFYMPKKATELKHLQCLEEELKPLEEVLNLAQSKNFHLEPRDLISNINVFVLELKGSETTFMCEYADETATIVEFLNRWITFSQSIISTLT

SEQ ID NO: 44 - protein, 132 aa, Artificial Sequence
  IL-2 analog 43
PTSSSTKKTQLQLEHLLLDLQMILNGINNYKNPKLTAMLTKKFYMPKKATELKHLQCLEEELKPLEEVLNLAQSKNFHLDPRDLISNINVLVLELKGSETTFMCEYADETATIVEFLNRWITFSQSIISTLT

SEQ ID NO: 45 - protein, 132 aa, Artificial Sequence
  IL-2 analog 44
PTSSSTKKTQLQLEHLLLDLQMILNGINNYKNPKLTAMLTKKFYMPKKATELKHLQCLEEELKPLEEVLNLAQSKNFHLDPRVLISNINVFVLELKGSETTFMCEYADETATIVEFLNRWITFSQSIISTLT

SEQ ID NO: 46 - protein, 132 aa, Artificial Sequence
  IL-2 analog 45
PTSSSTKKTQLQLEHLLLDLQMILNGINNYKNPKLTAMLTKKFYMPKKATELKHLQCLEEELKPLEEVLNLAQSKNFHLDPRFLISNINVFVLELKGSETTFMCEYADETATIVEFLNRWITFSQSIISTLT

SEQ ID NO: 47 - protein, 132 aa, Artificial Sequence
  IL-2 analog 46
PTSSSTKKTQLQLEHLLLVLQMILNGINNYKNPKLTAMLTKKFYMPKKATELKHLQCLEEELKPLEEVLNLAQSKNFHLDPRDLISNINVFVLELKGSETTFMCEYADETATIVEFLNRWITFSQSIISTLT

SEQ ID NO: 48 - protein, 132 aa, Artificial Sequence
  IL-2 analog 47
PTSSSTKKTQLQLEHLLLFLQMILNGINNYKNPKLTAMLTKKFYMPKKATELKHLQCLEEELKPLEEVLNLAQSKNFHLDPRDLISNINVFVLELKGSETTFMCEYADETATIVEFLNRWITFSQSIISTLT

SEQ ID NO: 49 - protein, 132 aa, Artificial Sequence
  IL-2 analog 48
PTSSSTKKTQLQLEHLLLDLQMILNGINNYKNPKLTAMLTKKFYMPKKATELKHLQCLEEELKPLEEVLNLAQSKNFHLDPRDLISVINVFVLELKGSETTFMCEYADETATIVEFLNRWITFSQSIISTLT

SEQ ID NO: 50 - protein, 132 aa, Artificial Sequence
  IL-2 analog 49
PTSSSTKKTQLQLEHLLLDLQMILNGINNYKNPKLTAMLTKKFYMPKKATELKHLQCLEEELKPLEEVLNLAQSKNFHLDPRDLISFINVFVLELKGSETTFMCEYADETATIVEFLNRWITFSQSIISTLT

SEQ ID NO: 51 - protein, 132 aa, Artificial Sequence
  IL-2 analog 50
PTSSSTKKTQLQLEHLLLDLQMILNGINNYKNPKLTRMLTKKFYMPKKATELKHLQCLEEELKPLEEVLNLAQSKNFHFDPRDVVSNINVFVLELKGSETTFMCEYADETATIVEFLNRWITFSQSIISTLT

SEQ ID NO: 52 - protein, 132 aa, Artificial Sequence
  IL-2 analog 51
PTSSSTKKTQLQLEHLLLDLQMILNGINNYKNPKLTRMLTFKFYMPKKATELKHLQCLEQELKPLEEVLNLAQSKNFHLDPRDLISNINVFVLELKGSETTFMCEYADETATIVEFLNRWITFSQSIISTLT

SEQ ID NO: 53 - protein, 132 aa, Artificial Sequence
  IL-2 analog 52
PTSSSTKKTQLQLEHLLLDLQMILNGINNYKNPKLTAMLTKKFYMPKKATELKHLQCLEEELKPLEEVLNLAQSKNFHFDPRDLISNINVFVLELKGSETTFMCEYADETATIVEFLNRWITFSQSIISTLT

SEQ ID NO: 54 - protein, 132 aa, Artificial Sequence
  IL-2 analog 53
PTSSSTKKTQLQLEHLLLDLQMILNGINNYKNPKLTAMLTKKFYMPKKATELKHLQCLEEELKPLEEVLNLAQSKNFHFDPRELISNINVFVLELKGSETTFMCEYADETATIVEFLNRWITFSQSIISTLT

SEQ ID NO: 55 - protein, 132 aa, Artificial Sequence
  IL-2 analog 54
PTSSSTKKTQLQLEHLLLDLQMILNGINNYKNPKLTAMLTKKFYMPKKATELKHLQCLEEELKPLEEVLNLAHSKNFHLDPRDLISNINVFVLELKGSETTFMCEYADETATIVEFLNRWITFSQSIISTLT

SEQ ID NO: 56 - protein, 132 aa, Artificial Sequence
  IL-2 analog 55
PTSSSTKKTQLQLEHLLLDLQMILNGINNYKNPKLTAMLTKKFYMPKKATELKHLQCLEEELKPLEEVLNLAHSKNFHFDPRDLISNINVFVLELKGSETTFMCEYADETATIVEFLNRWITFSQSIISTLT

SEQ ID NO: 57 - protein, 132 aa, Artificial Sequence
  IL-2 analog 56
PTSSSTKKTQLQLEHLLLDLQMILNGINNYKNPKLTAMLTKKFAMPKKATELKHLQCLEEELKPLEEVLNLAHSKNFHLDPRDLISNINVFVLELKGSETTFMCEYADETATIVEFLNRWITFSQSIISTLT

SEQ ID NO: 58 - protein, 132 aa, Artificial Sequence
  IL-2 analog 57
PTSSSTKKTQLQLEHLLLDLQMILNGINNYKNPKLTAMLTKKFAMPKKATELKHLQCLEEELKPLEEVLNLAHSKNFHFDPRDLISNINVFVLELKGSETTFMCEYADETATIVEFLNRWITFSQSIISTLT

SEQ ID NO: 59 - protein, 132 aa, Artificial Sequence
  IL-2 analog 61
PTSSSTKKTQLQLEHLLLDLQMILNGINNYKNPKLTAMLTKKFYMPKKATELKHLQCLEEELKPLEEVLNLAQSKNFHYDPRDGVSNINVYVLELKGSETTFMCEYADETATIVEFLNRWITFSQSIISTLT

SEQ ID NO: 60 - protein, 132 aa, Artificial Sequence
  IL-2 analog 59
PTSSSTKKTQLQLEHLLLDLQMILNGINNYKNPKLTAMLTKKFYMPKKATELKHLQCLEEELKPLEEVLNLAQSKNFHFDPRDAASNINVYVLELKGSETTFMCEYADETATIVEFLNRWITFSQSIISTLT

SEQ ID NO: 61 - protein, 132 aa, Artificial Sequence
  IL-2 analog 60
PTSSSTKKTQLQLEHLLLDLQMILNGINNYKNPKLTAMLTKKFAMPKKATELKHLQCLEEELKPLEEVLNLAQSKNFHYRPRDAASNINVYVLELKGSETTFMCEYADETATIVEFLNRWITFSQSIISTLT

SEQ ID NO: 62 - protein, 132 aa, Artificial Sequence; identical to SEQ ID NO: 59
  IL-2 analog 61

SEQ ID NO: 63 - protein, 132 aa, Artificial Sequence
  IL-2 analog 62
PTSSSTKKTQLQLEHLLLDLQMILNGINNYKNPKLTAMLTKKFYMPKKATELKHLQCLEEELKPLEEVLNLAQSKNFHWEPRDGASNINVFVLELKGSETTFMCEYADETATIVEFLNRWITFSQSIISTLT

SEQ ID NO: 64 - protein, 132 aa, Artificial Sequence
  IL-2 analog 63
PTSSSTKKTQLQLEHLLLDLQMILNGINNYKNPKLTAMLTKKFYMPKKATELKHLQCLEEELKPLEEVLNLAQSKNFHDEPRDTGSNINVFVLELKGSETTFMCEYADETATIVEFLNRWITFSQSIISTLT

SEQ ID NO: 65 - protein, 132 aa, Artificial Sequence
  IL-2 analog 64
PTSSSTKKTQLQLEHLLLDLQMILNGINNYKNPKLTAMLTKKFYMPKKATELKHLQCLEEELKPLEEVLNLAQSKNFHYNPRDVVSNINVYVLELKGSETTFMCEYADETATIVEFLNRWITFSQSIISTLT

SEQ ID NO: 66 - protein, 132 aa, Artificial Sequence
  IL-2 analog 65
PTSSSTKKTQLQLEHLLLDLQMILNGINNYKNPKLTAMLTKKFYMPKKATELKHLQCLEEELKPLEEVLNLAQSKNFHYEPRDVVSNINVFVLELKGSETTFMCEYADETATIVEFLNRWITFSQSIISTLT

SEQ ID NO: 67 - protein, 132 aa, Artificial Sequence
  IL-2 analog 66
PTSSSTKKTQLQLEHLLLDLQMILNGINNYKNPKLTAMLTKKFYMPKKATELKHLQCLEEELKPLEEVLNLAQSKNFHFEPRDFVSNINVFVLELKGSETTFMCEYADETATIVEFLNRWITFSQSIISTLT

SEQ ID NO: 68 - protein, 132 aa, Artificial Sequence
  IL-2 analog 67
PTSSSTKKTQLQLEHLLLDLQMILNGINNYKNPKLTAMLTKKFYMPKKATELKHLQCLEEELKPLEEVLNLAQSKNFHYDPRDFVSNINVWVLDLKGSETTFMCEYADETATIVEFLNRWITFSQSIISTLT

SEQ ID NO: 69 - protein, 132 aa, Artificial Sequence
  IL-2 analog 68
PTSSSTKKTQLQLEHLLLDLQMILNGINNYKNPKLTAMLTKKFYMPKKATELKHLQCLEEELKPLEEVLNLAQSKNFHFEPRDIVSNINEFVLELKGSETTFMCEYADETATIVEFLNRWITFSQSIISTLT

SEQ ID NO: 70 - protein, 132 aa, Artificial Sequence
  IL-2 analog 69
PTSSSTKKTQLQLEHLLLDLQMILNGINNYKNPKLTAMLTKKFYMPKKATELKHLQCLEEELKPLEEVLNLAQSKNFHYEPRDFLSNINEWVLDLKGSETTFMCEYADETATIVEFLNRWITFSQSIISTLT

SEQ ID NO: 71 - protein, 132 aa, Artificial Sequence
  IL-2 analog 70
PTSSSTKKTQLQLEHLLLDLQMILNGINNYKNPKLTAMLTKKFYMPKKATELKHLQCLEEELKPLEEVLNLAQSKNFHYDPRDVVSNINVFVLELKGSETTFMCEYADETATIVEFLNRWITFSQSIISTLT

SEQ ID NO: 72 - protein, 132 aa, Artificial Sequence
  IL-2 analog 71
PTSSSTKKTQLQLEHLLLDLQMILNGINNYKNPKLTAMLTKKFYMPKKATELKHLQCLEEELKPLEEVLNLAQSKNFHFEPRDVVSNINVFVLELKGSETTFMCEYADETATIVEFLNRWITFSQSIISTLT

SEQ ID NO: 73 - protein, 132 aa, Artificial Sequence
  IL-2 analog 72
PTSSSTKKTQLQLEHLLLDLQMILNGINNYKNPKLTAMLTKKFYMPKKATELKHLQCLEEELKPLEEVLNLAQSKNFHFDPRDVGSNINVFVLELKGSETTFMCEYADETATIVEFLNRWITFSQSIISTLT

SEQ ID NO: 74 - protein, 132 aa, Artificial Sequence
  IL-2 analog 73
PTSSSTKKTQLQLEHLLLDLQMILNGINNYKNPKLTAMLTKKFYMPKKATELKHLQCLEEELKPLEEVLNLAQSKNFHFDPRDWVSNINVFVLELKGSETTFMCEYADETATIVEFLNRWITFSQSIISTLT

SEQ ID NO: 75 - protein, 132 aa, Artificial Sequence
  IL-2 analog 74
PTSSSTKKTQLQLEHLLLDLQMILNGINNYKNPKLTDMLTKKFYMPKKATELKHLQCLEEELKPLEEVLNLAQSKNFHYDPRDVVSNINVFVLELKGSETTFMCEYADETATIVEFLNRWITFSQSIISTLT

SEQ ID NO: 76 - protein, 132 aa, Artificial Sequence
  IL-2 analog 75
PTSSSTKKTQLQLEHLLLDLQMILNGINNYKNPKLTAMLTKKFAMPKKATELKHLQCLEEELKPLEEVLNLAQSKNFHFEPRDVVSNINVFVLELKGSETTFMCEYADETATIVEFLNRWITFSQSIISTLT

SEQ ID NO: 77 - protein, 132 aa, Artificial Sequence
  IL-2 analog 76
PTSSSTKKTQLQLEHLLLDLQMILNGINNYKNPKLTAMLTKQFYMPKKATELKHLQCLERELKPLEEVLNLAQSKNFHFDPRDVGSNINVFVLELKGSETTFMCEYADETATIVEFLNRWITFSQSIISTLT

SEQ ID NO: 78 - protein, 132 aa, Artificial Sequence
  IL-2 analog 77
PTSSSTKKTQLQLEHLLLDLQMILNGINNYKNPKLTAMLTKEFYMPKKATELKHLQCLERELKPLEEVLNLAQSKNFHFDPRDWVSNINVFVLELKGSETTFMCEYADETATIVEFLNRWITFSQSIISTLT

SEQ ID NO: 79 - protein, 132 aa, Artificial Sequence
  IL-2 analog 78
PTSSSTKKTQLQLEHLLLDLQMILNGINNYKNPELTAMLTKKFYMPKKATELKHLQCLEEELKPLEEVLNLAQSKNFHFEPRDVVSNINVFVLELKGSETTFMCEYADETATIVEFLNRWITFSQSIISTLT

SEQ ID NO: 80 - protein, 132 aa, Artificial Sequence
  IL-2 analog 79
PTSSSTKKTQLQLEHLLLDLQMILNGINNYKNPELTAMLTKKFYMPKKATELKHLQCLEEELKPLEEVLNLAHSKNFHFEPRDVVSNINVFVLELKGSETTFMCEYADETATIVEFLNRWITFSQSIISTLT

SEQ ID NO: 81 - protein, 132 aa, Artificial Sequence
  IL-2 analog 80
PTSSSTKKTQLQLEHLLLDLQMILNGINNYKNPELTAMLTKKFYMPKKATELKHLQCLEEELKPLEEVLNLAHSKNFHFEGRDVVSNINVFVLELKGSETTFMCEYADETATIVEFLNRWITFSQSIISTLT

SEQ ID NO: 82 - protein, 132 aa, Artificial Sequence
  IL-2 analog 81
PTSSSTKKTQLQLEHLLLDLQMILNGINNYKNPELTAMLTKKFYMPKKATELKHLQCLEEELKPLEEVLNLAHSKNFHFEVRDVVSNINVFVLELKGSETTFMCEYADETATIVEFLNRWITFSQSIISTLT

SEQ ID NO: 83 - protein, 132 aa, Artificial Sequence
  IL-2 analog 82
PTSSSTKKTQLQLEHLRLDLEMILNGINNYKNPKLTRMLTFKFYMPKKATELKHLQCLEEELKPLEEVLNLAQSKNFHFDPRDEVSNINVFVLELKGSETTFMCEYADETATIVEFLNRWITFSQSIISTLT

SEQ ID NO: 84 - protein, 132 aa, Artificial Sequence
  IL-2 analog 83
PTSSSTKKTQLQLEHLRRDLEMILNGINNYKNPKLTRMLTFKFYMPKKATELKHLQCLEEELKPLEEVLNLAQSKNFHFDPRDEVSNINVFVLELKGSETTFMCEYADETATIVEFLNRWITFSQSIISTLT

SEQ ID NO: 85 - protein, 132 aa, Artificial Sequence
  IL-2 analog 84
PTSSSTKKTQLQLEHLRLDLEMILNGINNYKNPKLTRMLTFKFYMPKKATELKHLQCLEEELKPLEEVLNLAQSKNFHVDPRDEVSNINVFVLELKGSETTFMCEYADETATIVEFLNRWITFSQSIISTLT

SEQ ID NO: 86 - protein, 132 aa, Artificial Sequence
  IL-2 analog 85
PTSSSTKKTQLQLEHLLLDLQMILNGINNYKNPKLTRMLTFKFYMPKKATELKHLQCLEEELKPLEEVLNLAQSKNFHFEPRDVVSNINVFVLELKGSETTFMCEYADETATIVEFLNRWITFSQSIISTLT

SEQ ID NO: 87 - protein, 132 aa, Artificial Sequence
  IL-2 analog 86
PTSSSTKKTQLQLEHLRLDLEMILNGINNYKNPKLTRMLTFKFYMPKKATELKHLQCLEEELKPLEEVLNLAQSKNFHFEPRDVVSNINVFVLELKGSETTFMCEYADETATIVEFLNRWITFSQSIISTLT

SEQ ID NO: 88 - protein, 132 aa, Artificial Sequence
  IL-2 analog 87
PTSSSTKKTQLQLEHLRRDLEMILNGINNYKNPKLTRMLTFKFYMPKKATELKHLQCLEEELKPLEEVLNLAQSKNFHFEPRDVVSNINVFVLELKGSETTFMCEYADETATIVEFLNRWITFSQSIISTLT

SEQ ID NO: 89 - protein, 132 aa, Artificial Sequence
  IL-2 analog 88
PTSSSTKKTQLQLEHLLLDLQMILNGINNYKNPKLTRMLTFKFYMPKKATELKHLQCLEDELKPLEEVLNLAQSKNFHFEPRDVVSNINVFVLELKGSETTFMCEYADETATIVEFLNRWITFSQSIISTLT

SEQ ID NO: 90 - protein, 132 aa, Artificial Sequence
  IL-2 analog 89
PTSSSTKKTQLQLEHLLLDLQMILNGINNYKNPKLTAMLTFKFYMPKKATELKHLQCLEEELKPLEQVLNLAQSKNFHFEPRDVVSNINVFVLELKGSETTFMCEYADETATIVEFLNRWITFSQSIISTLT

SEQ ID NO: 91 - protein, 132 aa, Artificial Sequence
  IL-2 analog 90
PTSSSTKKTQLQLEHLLLDLQMILNGINNYKNPKLTRMLTWKFYMPKKATELKHLQCLEEELKPLEEVLNLAQSKNFHFEPRDVVSNINVFVLELKGSETTFMCEYADETATIVEFLNRWITFSQSIISTLT

SEQ ID NO: 92 - protein, 132 aa, Artificial Sequence
  IL-2 analog 91
PTSSSTKKTQLQLEHLLLDLQMILNGINNYKNPKLTRMLTFKFYMPKKATELKHLQCLEQELKPLEEVLNLAQSKNFHFEPRDVVSNINVFVLELKGSETTFMCEYADETATIVEFLNRWITFSQSIISTLT

SEQ ID NO: 93 - protein, 132 aa, Artificial Sequence
  IL-2 analog 92
PTSSSTKKTQLQLEHLLLDLQMILNGINNYKNPKLTRMLTFKFYMPKKATELKHLQCLEEELKPLEEVLNLAQSKNFHFEPRDVVSNINTFVLELKGSETTFMCEYADETATIVEFLNRWITFSQSIISTLT

SEQ ID NO: 94 - protein, 132 aa, Artificial Sequence
  IL-2 analog 93
PTSSSTKKTQLQLEHLLLDLQMILNGINNYKNPKLTRMLTFKFYMPKKATELKHLQCLEEELKPLEEVLNLAQSKNFHFEPREVVSNINTFVLELKGSETTFMCEYADETATIVEFLNRWITFSQSIISTLT

SEQ ID NO: 95 - protein, 132 aa, Artificial Sequence
  IL-2 analog 94
PTSSSTKKTQLQLEHLLLDLQMILNGINNYKNPKLTRMLTFKFYMPKKATELKHLQCLEEELKPLEEVLNLAQSKNFHFEPRDVVSNINVFVFEFKGSETTFMCEYADETATIVEFLNRWITFSQSIISTLT

SEQ ID NO: 96 - protein, 132 aa, Artificial Sequence
  IL-2 analog 95
PTSSSTKKTQLQLEHLLLDLQMILNGINNYKNPKLTRMLTFKFYMPKKATELKHLQCLEEELKPLEEGLNLAQSKNFHFEPRDVVSNINVFVLELKGSETTFMCEYADETATIVEFLNRWITFSQSIISTLT

SEQ ID NO: 97 - protein, 132 aa, Artificial Sequence
  IL-2 analog 96
PTSSSTKKTQLQLEHLLLDLQMILNGINNYKNPKLTRMLTFKFYMPKKATELKHLQCLEEELKPLEEGLNLAASKNFHFEPRDVVSNINVFVLELKGSETTFMCEYADETATIVEFLNRWITFSQSIISTLT

SEQ ID NO: 98 - protein, 132 aa, Artificial Sequence
  IL-2 analog 97
PTSSSTKKTQLQLEHLLLDLQMILNGINNYKNPKLTAMLTFKFYMPKKATELKHLQCLEEELKPLEEVLNLAQSKNFHFDPRDLISNINVFVLELKGSETTFMCEYADETATIVEFLNRWITFSQSIISTLT

SEQ ID NO: 99 - protein, 132 aa, Artificial Sequence
  IL-2 analog 98
PTSSSTKKTQLQLEHLLLDLQMILNGINNYKNPKLTAMLTFKFYMPKKATELKHLQCLEEELKPLEEVLNLAQSKNFHFEPRDVISNINVFVLELKGSETTFMCEYADETATIVEFLNRWITFSQSIISTLT

SEQ ID NO: 100 - protein, 132 aa, Artificial Sequence
  IL-2 analog 99
PTSSSTKKTQLQLEHLLLDLQMILNGINNYKNPKLTAMLTFKFYMPKKATELKHLQCLEEELKPLEEVLNLAQSKNFHFEPRDLVSNINVFVLELKGSETTFMCEYADETATIVEFLNRWITFSQSIISTLT

SEQ ID NO: 101 - protein, 132 aa, Artificial Sequence
  IL-2 analog 100
PTSSSTKKTQLQLEHLLLDLQMILNGINNYKNPKLTRMLTFKFYMPKKATELKHLQCLEEELKPLEEVLNLAQSKNFHFEPRDYVSNINVFVLELKGSETTFMCEYADETATIVEFLNRWITFSQSIISTLT

SEQ ID NO: 102 - protein, 132 aa, Artificial Sequence
  IL-2 analog 101
PTSSSTKKTQLQLEHLLLDLQMILNGINNYKNPKLTRMLTFKFYMPKKATELKHLQCLEEELKPLEEVLNLAQSKNFHFEPRDLASNINVFVLELKGSETTFMCEYADETATIVEFLNRWITFSQSIISTLT

SEQ ID NO: 103 - protein, 132 aa, Artificial Sequence
  IL-2 analog 102
PTSSSTKKTQLQLEHLLLDLQMILNGINNYKNPKLTRMLTFKFYMPKKATELKHLQCLEEELKPLEEVLNLAQSKNFHFEPRDVVSNINVIVLELKGSETTFMCEYADETATIVEFLNRWITFSQSIISTLT

SEQ ID NO: 104 - protein, 132 aa, Artificial Sequence
  IL-2 analog 103
PTSSSTKKTQLQLEHLRLDLEMILNGINNYKNPKLTAMLTFKFYMPKKATELKHLQCLEEELKPLEEVLNLAQSKNFHFEPRDVVSNINVFVLELKGSETTFMCEYADETATIVEFLNRWITFSQSIISTLT

SEQ ID NO: 105 - protein, 132 aa, Artificial Sequence
  IL-2 analog 104
PTSSSTKKTQLQLEHLRLDLEMILNGINNYKNPKLTRMLTFKFYMPKKATELKHLQCLEDELKPLEEVLNLAQSKNFHFEPRDVVSNINVFVLELKGSETTFMCEYADETATIVEFLNRWITFSQSIISTLT

SEQ ID NO: 106 - protein, 132 aa, Artificial Sequence
  IL-2 analog 105
PTSSSTKKTQLQLEHLRLDLEMILNGINNYKNPKLTRMLTFKFYMPKKATELKHLQCLEEELKPLEDVLNLAQSKNFHFEPRDVVSNINVFVLELKGSETTFMCEYADETATIVEFLNRWITFSQSIISTLT

SEQ ID NO: 107 - DNA, 399 bp, Artificial Sequence
  IL-2 analog 1
cctacttcaagttctacaaagaaaacacagctacaactggagcatttactgctggatttacagatgattttgaatggaattaataattacaagaatcccaaactcaccaggatgctcacatttaagttttacatgcccaagaaggccacagaactgaaacatcttcagtgtctagaagaagaactcaaacctctggaggaagtgctaaatttagctcaaagcaaaaactttcacttaagacccagggacttaatcagcaatatcaacgtaatagttctggaactaaagggatctgaaacaacattcatgtgtgaatatgctgatgagacagcaaccattgtagaatttctgaacagatggattacctttagtcaaagcatcatctcaacactgacttga

SEQ ID NO: 108 - DNA, 399 bp, Artificial Sequence
  IL-2 analog 2
cctacttcaagttctacaaagaaaacacagctacaactggagcatttactgctggatttacagatgattttgaatggaattaataattacaagaatcccaaactcaccaggatgctcacatttaagttttacatgcccaagaaggccacagaactgaaacatcttcagtgtctagaagaagaactcaaacctctggaggaagtgctaaatttagctcaaagcaaaaactttcacttaagacccagggacttaatctgcaatatcaacgtaatagttctggaactaaagggatctgaaacaacattcatgtgtgaatatgctgatgagacagcaaccattgtagaatttctgaacagatggattacctttagtcaaagcatcatctcaacactgacttga

SEQ ID NO: 109 - DNA, 399 bp, Artificial Sequence
  IL-2 analog 3
cctacttcaagttctacaaagaaaacacagctacaactggagcatttactgctggatttacagatgattttgaatggaattaataattactgtaatcccaaactcaccaggatgctcacatttaagttttacatgcccaagaaggccacagaactgaaacatcttcagtgtctagaagaagaactcaaacctctggaggaagtgctaaatttagctcaaagcaaaaactttcacttaagacccagggacttaatcagcaatatcaacgtaatagttctggaactaaagggatctgaaacaacattcatgtgtgaatatgctgatgagacagcaaccattgtagaatttctgaacagatggattacctttagtcaaagcatcatctcaacactgacttga

SEQ ID NO: 110 - DNA, 399 bp, Artificial Sequence
  IL-2 analog 4
cctacttcaagttctacaaagaaaacacagctacaactggagcatttactgctggatttacagatgattttgaatggaattaataattacaagaatccctgtctcaccaggatgctcacatttaagttttacatgcccaagaaggccacagaactgaaacatcttcagtgtctagaagaagaactcaaacctctggaggaagtgctaaatttagctcaaagcaaaaactttcacttaagacccagggacttaatcagcaatatcaacgtaatagttctggaactaaagggatctgaaacaacattcatgtgtgaatatgctgatgagacagcaaccattgtagaatttctgaacagatggattacctttagtcaaagcatcatctcaacactgacttga

SEQ ID NO: 111 - DNA, 399 bp, Artificial Sequence
  IL-2 analog 5
cctacttcaagttctacaaagaaaacacagctacaactggagcatttactgctggatttacagatgattttgaatggaattaataattacaagaatcccaaactcaccaggatgctcacattttgtttttacatgcccaagaaggccacagaactgaaacatcttcagtgtctagaagaagaactcaaacctctggaggaagtgctaaatttagctcaaagcaaaaactttcacttaagacccagggacttaatcagcaatatcaacgtaatagttctggaactaaagggatctgaaacaacattcatgtgtgaatatgctgatgagacagcaaccattgtagaatttctgaacagatggattacctttagtcaaagcatcatctcaacactgacttga

SEQ ID NO: 112 - DNA, 399 bp, Artificial Sequence
  IL-2 analog 6
cctacttcaagttctacaaagaaaacacagctacaactggagcatttactgctggatttacagatgattttgaatggaattaataattacaagaatcccaaactcaccaggatgctcacatttaagttttacatgccctgtaaggccacagaactgaaacatcttcagtgtctagaagaagaactcaaacctctggaggaagtgctaaatttagctcaaagcaaaaactttcacttaagacccagggacttaatcagcaatatcaacgtaatagttctggaactaaagggatctgaaacaacattcatgtgtgaatatgctgatgagacagcaaccattgtagaatttctgaacagatggattacctttagtcaaagcatcatctcaacactgacttga

SEQ ID NO: 113 - DNA, 399 bp, Artificial Sequence
  IL-2 analog 7
cctacttcaagttctacaaagaaaacacagctacaactggagcatttactgctggatttacagatgattttgaatggaattaataattacaagaatcccaaactcaccaggatgctcacatttaagttttacatgcccaagtgtgccacagaactgaaacatcttcagtgtctagaagaagaactcaaacctctggaggaagtgctaaatttagctcaaagcaaaaactttcacttaagacccagggacttaatcagcaatatcaacgtaatagttctggaactaaagggatctgaaacaacattcatgtgtgaatatgctgatgagacagcaaccattgtagaatttctgaacagatggattacctttagtcaaagcatcatctcaacactgacttga

SEQ ID NO: 114 - DNA, 399 bp, Artificial Sequence
  IL-2 analog 8
cctacttcaagttctacaaagaaaacacagctacaactggagcatttactgctggatttacagatgattttgaatggaattaataattacaagaatcccaaactcaccaggatgctcacatttaagttttacatgcccaagaaggccacagaactgaaacatcttcagtgtctagaagaagaactcaaacctctggaggaagtgctaaatttagctcaaagctgtaactttcacttaagacccagggacttaatcagcaatatcaacgtaatagttctggaactaaagggatctgaaacaacattcatgtgtgaatatgctgatgagacagcaaccattgtagaatttctgaacagatggattacctttagtcaaagcatcatctcaacactgacttga

SEQ ID NO: 115 - DNA, 399 bp, Artificial Sequence
  IL-2 analog 9
cctacttcaagttctacaaagaaaacacagctacaactggagcatttactgctggatttacagatgattttgaatggaattaataattacaagaatcccaaactcaccgcgatgctcacatttaagttttacatgcccaagaaggccacagaactgaaacatcttcagtgtctagaagaagaactcaaacctctggaggaagtgctaaatttagctcaaagcaaaaactttcacttaagacccagggacttaatcagcaatatcaacgtaatagttctggaactaaagggatctgaaacaacattcatgtgtgaatatgctgatgagacagcaaccattgtagaatttctgaacagatggattacctttagtcaaagcatcatctcaacactgacttga

SEQ ID NO: 116 - DNA, 399 bp, Artificial Sequence
  IL-2 analog 10
cctacttcaagttctacaaagaaaacacagctacaactggagcatttactgctggatttacagatgattttgaatggaattaataattacaagaatcccaaactcaccaggatgctcacaaagaagttttacatgcccaagaaggccacagaactgaaacatcttcagtgtctagaagaagaactcaaacctctggaggaagtgctaaatttagctcaaagcaaaaactttcacttaagacccagggacttaatcagcaatatcaacgtaatagttctggaactaaagggatctgaaacaacattcatgtgtgaatatgctgatgagacagcaaccattgtagaatttctgaacagatggattacctttagtcaaagcatcatctcaacactgacttga

SEQ ID NO: 117 - DNA, 399 bp, Artificial Sequence
  IL-2 analog 11
cctacttcaagttctacaaagaaaacacagctacaactggagcatttactgctggatttacagatgattttgaatggaattaataattacaagaatcccaaactcaccaggatgctcacagctaagttttacatgcccaagaaggccacagaactgaaacatcttcagtgtctagaagaagaactcaaacctctggaggaagtgctaaatttagctcaaagcaaaaactttcacttaagacccagggacttaatcagcaatatcaacgtaatagttctggaactaaagggatctgaaacaacattcatgtgtgaatatgctgatgagacagcaaccattgtagaatttctgaacagatggattacctttagtcaaagcatcatctcaacactgacttga

SEQ ID NO: 118 - DNA, 399 bp, Artificial Sequence
  IL-2 analog 12
cctacttcaagttctacaaagaaaacacagctacaactggagcatttactgctggatttacagatgattttgaatggaattaataattacaagaatcccaaactcaccgcgatgctcacaaagaagttttacatgcccaagaaggccacagaactgaaacatcttcagtgtctagaagaagaactcaaacctctggaggaagtgctaaatttagctcaaagcaaaaactttcacttaagacccagggacttaatcagcaatatcaacgtaatagttctggaactaaagggatctgaaacaacattcatgtgtgaatatgctgatgagacagcaaccattgtagaatttctgaacagatggattacctttagtcaaagcatcatctcaacactgacttga

SEQ ID NO: 119 - DNA, 399 bp, Artificial Sequence
  IL-2 analog 13
cctacttcaagttctacaaagaaaacacagctacaactggagcatttactgctggatttacagatgattttgaatggaattaataattacaagaatcccaaactcaccgcgatgctcacagctaagttttacatgcccaagaaggccacagaactgaaacatcttcagtgtctagaagaagaactcaaacctctggaggaagtgctaaatttagctcaaagcaaaaactttcacttaagacccagggacttaatcagcaatatcaacgtaatagttctggaactaaagggatctgaaacaacattcatgtgtgaatatgctgatgagacagcaaccattgtagaatttctgaacagatggattacctttagtcaaagcatcatctcaacactgacttga

SEQ ID NO: 120 - DNA, 399 bp, Artificial Sequence
  IL-2 analog 14
cctacttcaagttctacaaagaaaacacagctacaactggagcatttactgtacgatttacagatgattttgaatggaattaataattacaagaatcccaaactcaccgcgatgctcacaaagaagttttacatgcccaagaaggccacagaactgaaacatcttcagtgtctagaagaagaactcaaacctctggaggaagtgctaaatttagctcaaagcaaaaactttcacttaagacccagggacttaatcagcaatatcaacgtaatagttctggaactaaagggatctgaaacaacattcatgtgtgaatatgctgatgagacagcaaccattgtagaatttctgaacagatggattacctttagtcaaagcatcatctcaacactgacttga

SEQ ID NO: 121 - DNA, 399 bp, Artificial Sequence
  IL-2 analog 15
cctacttcaagttctacaaagaaaacacagctacaactggagcatttactgctggatttacagatgattttgaatggaattaataattacaagaatcccaaactcaccgcgatgctcacaaagaagttttacatgcccaagaaggccacagaactgaaacatcttcagtgtctagaagaagaactcaaacctctggaggaagtgctaaatttagctcaaagcaaaaactttcacttaagacccagggagttaatcagcaatatcaacgtaatagttctggaactaaagggatctgaaacaacattcatgtgtgaatatgctgatgagacagcaaccattgtagaatttctgaacagatggattacctttagtcaaagcatcatctcaacactgacttga

SEQ ID NO: 122 - DNA, 399 bp, Artificial Sequence
  IL-2 analog 16
cctacttcaagttctacaaagaaaacacagctacaactggagcatttactgctggatttacagatgattttgaatggaattaataattacaagaatcccaaactcaccgcgatgctcacaaagaagttttacatgcccaagaaggccacagaactgaaacatcttcagtgtctagaagaagaactcaaacctctggaggaagtgctaaatttagctcaaagcaaaaactttcacttaagacccagggacttaatcagccaaatcaacgtaatagttctggaactaaagggatctgaaacaacattcatgtgtgaatatgctgatgagacagcaaccattgtagaatttctgaacagatggattacctttagtcaaagcatcatctcaacactgacttga

SEQ ID NO: 123 - DNA, 399 bp, Artificial Sequence
  IL-2 analog 17
cctacttcaagttctacaaagaaaacacagctacaactggagcatttactgctggatttacagatgattttgaatggaattaataattacaagaatcccaaactcaccgcgatgctcacaaagaagttttacatgcccaagaaggccacagaactgaaacatcttcagtgtctagaagaagaactcaaacctctggaggaagtgctaaatttagctcaaagcaaaaactttcacttaagacccagggacttaatcagcaatatcaacacaatagttctggaactaaagggatctgaaacaacattcatgtgtgaatatgctgatgagacagcaaccattgtagaatttctgaacagatggattacctttagtcaaagcatcatctcaacactgacttga

SEQ ID NO: 124 - DNA, 399 bp, Artificial Sequence
  IL-2 analog 18
cctacttcaagttctacaaagaaaacacagctacaactggagcatttactgctggatttacagatgattttgaatggaattaataattacaagaatcccaaactcaccgcgatgctcacaaagaagttttacatgcccaagaaggccacagaactgaaacatcttcagtgtctagaacaggaactcaaacctctggaggaagtgctaaatttagctcaaagcaaaaactttcacttaagacccagggacttaatcagcaatatcaacgtaatagttctggaactaaagggatctgaaacaacattcatgtgtgaatatgctgatgagacagcaaccattgtagaatttctgaacagatggattacctttagtcaaagcatcatctcaacactgacttga

SEQ ID NO: 125 - DNA, 399 bp, Artificial Sequence
  IL-2 analog 19
cctacttcaagttctacaaagaaaacacagctacaactggagcatttactgctggatttacagatgattttgaatggaattaataattacaagaatcccaaactcaccgcgatgctcacaaagaagttttacatgcccaagaaggccacagaactgaaacatcttcagtgtctagaagaagaactcaaacctctggaggaagtgctaaatttagctcaaagcaaaaactttcacttagaccccagggacttaatcagcaatatcaacgtatttgttctggaactaaagggatctgaaacaacattcatgtgtgaatatgctgatgagacagcaaccattgtagaatttctgaacagatggattacctttagtcaaagcatcatctcaacactgacttga

SEQ ID NO: 126 - DNA, 399 bp, Artificial Sequence
  IL-2 analog 20
cctacttcaagttctacaaagaaaacacagctacaactggagcatttactgctggatttacagatgattttgaatggaattaataattacaagaatcccaaactcaccgcgatgctcacaaagaagttttacatgcccaagaaggccacagaactgaaacatcttcagtgtctagaagaagaactcaaacctctggaggaagtgctaaatttagctcaaagcaaaaactttcacttaagacccagggacgtagtcagcaatatcaacgtatttgttctggaactaaagggatctgaaacaacattcatgtgtgaatatgctgatgagacagcaaccattgtagaatttctgaacagatggattacctttagtcaaagcatcatctcaacactgacttga

SEQ ID NO: 127 - DNA, 399 bp, Artificial Sequence
  IL-2 analog 21
cctacttcaagttctacaaagaaaacacagctacaactggagcatttactgctggatttacagatgattttgaatggaattaataattacaagaatcccaaactcaccgcgatgctcacaaagaagttttacatgcccaagaaggccacagaactgaaacatcttcagtgtctagaagaagaactcaaacctctggaggaagtgctaaatttagctcaaagcaaaaactttcactttgaccccagggacgtagtcagcaatatcaacgtatttgttctggaactaaagggatctgaaacaacattcatgtgtgaatatgctgatgagacagcaaccattgtagaatttctgaacagatggattacctttagtcaaagcatcatctcaacactgacttga

SEQ ID NO: 128 - DNA, 399 bp, Artificial Sequence
  IL-2 analog 22
cctacttcaagttctacaaagaaaacacaggtacaactggagcatttactgctggatttacagatgattttgaatggaattaataattacaagaatcccaaactcaccgcgatgctcacaaagaagttttacatgcccaagaaggccacagaactgaaacatcttcagtgtctagaagaagaactcaaacctctggaggaagtgctaaatttagctcaaagcaaaaactttcacttaagacccagggacttaatcagcaatatcaacgtaatagttctggaactaaagggatctgaaacaacattcatgtgtgaatatgctgatgagacagcaaccattgtagaatttctgaacagatggattacctttagtcaaagcatcatctcaacactgacttga

SEQ ID NO: 129 - DNA, 399 bp, Artificial Sequence
  IL-2 analog 23
cctacttcaagttctacaaagaaaacacagtttcaactggagcatttactgctggatttacagatgattttgaatggaattaataattacaagaatcccaaactcaccgcgatgctcacaaagaagttttacatgcccaagaaggccacagaactgaaacatcttcagtgtctagaagaagaactcaaacctctggaggaagtgctaaatttagctcaaagcaaaaactttcacttaagacccagggacttaatcagcaatatcaacgtaatagttctggaactaaagggatctgaaacaacattcatgtgtgaatatgctgatgagacagcaaccattgtagaatttctgaacagatggattacctttagtcaaagcatcatctcaacactgacttga

SEQ ID NO: 130 - DNA, 399 bp, Artificial Sequence
  IL-2 analog 24
cctacttcaagttctacaaagaaaacacagctacaactggagcatttactggtggatttacagatgattttgaatggaattaataattacaagaatcccaaactcaccgcgatgctcacaaagaagttttacatgcccaagaaggccacagaactgaaacatcttcagtgtctagaagaagaactcaaacctctggaggaagtgctaaatttagctcaaagcaaaaactttcacttaagacccagggacttaatcagcaatatcaacgtaatagttctggaactaaagggatctgaaacaacattcatgtgtgaatatgctgatgagacagcaaccattgtagaatttctgaacagatggattacctttagtcaaagcatcatctcaacactgacttga

SEQ ID NO: 131 - DNA, 399 bp, Artificial Sequence
  IL-2 analog 25
cctacttcaagttctacaaagaaaacacagctacaactggagcatttactgttcgatttacagatgattttgaatggaattaataattacaagaatcccaaactcaccgcgatgctcacaaagaagttttacatgcccaagaaggccacagaactgaaacatcttcagtgtctagaagaagaactcaaacctctggaggaagtgctaaatttagctcaaagcaaaaactttcacttaagacccagggacttaatcagcaatatcaacgtaatagttctggaactaaagggatctgaaacaacattcatgtgtgaatatgctgatgagacagcaaccattgtagaatttctgaacagatggattacctttagtcaaagcatcatctcaacactgacttga

SEQ ID NO: 132 - DNA, 399 bp, Artificial Sequence
  IL-2 analog 26
cctacttcaagttctacaaagaaaacacagctacaactggagcatttactgctggatttacagatgattttgaatggaattaataattacaagaatcccaaactcaccgcgatgctcacaaagaagttttacatgcccaagaaggccacagaactgaaacatcttcagtgtctagaagaagaactcaaacctctggaggaagtgctaaatttagctcaaagcaaaaactttcacttaagacccagggacttaatcagcaatttcaacgtaatagttctggaactaaagggatctgaaacaacattcatgtgtgaatatgctgatgagacagcaaccattgtagaatttctgaacagatggattacctttagtcaaagcatcatctcaacactgacttga

SEQ ID NO: 133 - DNA, 399 bp, Artificial Sequence
  IL-2 analog 27
cctacttcaagttctacaaagaaaacacagctacaactggagcatttactgctggatttacagatgattttgaatggaattaataattacaagaatcccaaactcaccgcgatgctcacaaagaagttttacatgcccaagaaggccacagaactgaaacatcttcagtgtctagaagaagaactcaaacctctggaggaagtgctaaatttagctcaaagcaaaaactttcacttaagacccagggacttaatcagcaatatcaactttatagttctggaactaaagggatctgaaacaacattcatgtgtgaatatgctgatgagacagcaaccattgtagaatttctgaacagatggattacctttagtcaaagcatcatctcaacactgacttga

SEQ ID NO: 134 - DNA, 399 bp, Artificial Sequence
  IL-2 analog 28
cctacttcaagttctacaaagaaaacacagctacaactggagcatttactgctggatttacagatgattttgaatggaattaataattacaagaatcccaaactcaccgcgatgctcacaaagaagttttacatgcccaagaaggccacagaactgaaacatcttcagtgtctagaagaagaactcaaacctctggaggaagtgctaaatttagctcaaagcaaaaactttcacttaagacccagggacttaatcagcaatatcaacgtaatagttgtggaactaaagggatctgaaacaacattcatgtgtgaatatgctgatgagacagcaaccattgtagaatttctgaacagatggattacctttagtcaaagcatcatctcaacactgacttga

SEQ ID NO: 135 - DNA, 399 bp, Artificial Sequence
  IL-2 analog 29
cctacttcaagttctacaaagaaaacacagctacaactggagcatttactgctggatttacagatgattttgaatggaattaataattacaagaatcccaaactcaccgcgatgctcacaaagaagttttacatgcccaagaaggccacagaactgaaacatcttcagtgtctagaagaagaactcaaacctctggaggaagtgctaaatttagctcaaagcaaaaactttcacttaagacccagggacttaatcagcaatatcaacgtaatagttctggaactaaagggatctgaaacaacattcatgtgtgaatatgctgatgagacagcaaccattgtagaatttctgaacagatggattacctttagtacaagcatcatctcaacactgacttga

SEQ ID NO: 136 - DNA, 399 bp, Artificial Sequence
  IL-2 analog 30
cctacttcaagttctacaaagaaaacacagctacaactggagcatttactgctggatttacagatgattttgaatggaattaataattacaagaatcccaaactcaccgcgatgctcacatttaagttttacatgcccaagaaggccacagaactgaaacatcttcagtgtctagaagaagaactcaaacctctggaggaagtgctaaatttagctcaaagcaaaaactttcacttagaccccagggacttaatcagcaatatcaacgtatttgttctggaactaaagggatctgaaacaacattcatgtgtgaatatgctgatgagacagcaaccattgtagaatttctgaacagatggattacctttagtcaaagcatcatctcaacactgacttga

SEQ ID NO: 137 - DNA, 399 bp, Artificial Sequence
  IL-2 analog 31
cctacttcaagttctacaaagaaaacacagctacaactggagcatttactgctggatttacagatgattttgaatggaattaataattacaagaatcccaaactcaccgcgatgctcacatttaagttttacatgcccaagaaggccacagaactgaaacatcttcagtgtctagaagaagaactcaaacctctggaggaagtgctaaatttagctcaaagcaaaaactttcacttaagacccagggagttaatcagcaatatcaacgtaatagttctggaactaaagggatctgaaacaacattcatgtgtgaatatgctgatgagacagcaaccattgtagaatttctgaacagatggattacctttagtcaaagcatcatctcaacactgacttga

SEQ ID NO: 138 - DNA, 399 bp, Artificial Sequence
  IL-2 analog 32
cctacttcaagttctacaaagaaaacacagctacaactggagcatttactgctggatttacagatgattttgaatggaattaataattacaagaatcccaaactcaccgcgatgctcacatttaagttttacatgcccaagaaggccacagaactgaaacatcttcagtgtctagaagaagaactcaaacctctggaggaagtgctaaatttagctcaaagcaaaaactttcacttagaccccagggagttaatcagcaatatcaacgtatttgttctggaactaaagggatctgaaacaacattcatgtgtgaatatgctgatgagacagcaaccattgtagaatttctgaacagatggattacctttagtcaaagcatcatctcaacactgacttga

SEQ ID NO: 139 - DNA, 399 bp, Artificial Sequence
  IL-2 analog 33
cctacttcaagttctacaaagaaaacacagctacaactggagcatttactgctggatttacagatgattttgaatggaattaataattacaagaatcccaaactcaccgcgatgctcacatttaagttttacatgcccaagaaggccacagaactgaaacatcttcagtgtctagaagaagaactcaaacctctggaggaagtgctaaatttagctcaaagcaaaaactttcactttagacccagggacttaatcagcaatatcaacgtaatagttctggaactaaagggatctgaaacaacattcatgtgtgaatatgctgatgagacagcaaccattgtagaatttctgaacagatggattacctttagtcaaagcatcatctcaacactgacttga

SEQ ID NO: 140 - DNA, 399 bp, Artificial Sequence
  IL-2 analog 34
cctacttcaagttctacaaagaaaacacagctacaactggagcatttactgctggatttacagatgattttgaatggaattaataattacaagaatcccaaactcaccgcgatgctcacatttaagttttacatgcccaagaaggccacagaactgaaacatcttcagtgtctagaagaagaactcaaacctctggaggaagtgctaaatttagctcaaagcaaaaactttcactttagacccagggagttaatcagcaatatcaacgtaatagttctggaactaaagggatctgaaacaacattcatgtgtgaatatgctgatgagacagcaaccattgtagaatttctgaacagatggattacctttagtcaaagcatcatctcaacactgacttga

SEQ ID NO: 141 - DNA, 399 bp, Artificial Sequence
  IL-2 analog 35
cctacttcaagttctacaaagaaaacacagctacaactggagcatttactgctggatttacagatgattttgaatggaattaataattacaagaatcccaaactcaccgcgatgctcacatttaagttttacatgcccaagaaggccacagaactgaaacatcttcagtgtctagaagaagaactcaaacctctggaggaagtgctaaatttagctcaaagcaaaaactttcacttaagacccagggacttaatcagcaatatcaacgtaatagttttcgaatttaagggatctgaaacaacattcatgtgtgaatatgctgatgagacagcaaccattgtagaatttctgaacagatggattacctttagtcaaagcatcatctcaacactgacttga

SEQ ID NO: 142 - DNA, 399 bp, Artificial Sequence
  IL-2 analog 36
cctacttcaagttctacaaagaaaacacagctacaactggagcatttactgctggatttacagatgattttgaatggaattaataattacaagaatcccaaactcaccgcgatgctcacatttaagttttacatgcccaagaaggccacagaactgaaacatcttcagtgtctagaagaagaactcaaacctctggaggaagtgctaaatttagctcaaagcaaaaactttcacttaagacccagggacttaatcagcaatatcaacgtaatagttttcgaagtaaagggatctgaaacaacattcatgtgtgaatatgctgatgagacagcaaccattgtagaatttctgaacagatggattacctttagtcaaagcatcatctcaacactgacttga

SEQ ID NO: 143 - DNA, 399 bp, Artificial Sequence
  IL-2 analog 37
cctacttcaagttctacaaagaaaacacagctacaactggagcatttactgctggatttacagatgattttgaatggaattaataattacaagaatcccaaactcaccgcgatgctcacaaagaagttttacatgcccaagaaggccacagaactgaaacatcttcagtgtctagaagaagaactcaaacctctggaggaagtgctaaatttagctcaaagcaaaaactttcacttagaccccagggacttaatcagcaatatcaacgtattagttctggaactaaagggatctgaaacaacattcatgtgtgaatatgctgatgagacagcaaccattgtagaatttctgaacagatggattacctttagtcaaagcatcatctcaacactgacttga

SEQ ID NO: 144 - DNA, 399 bp, Artificial Sequence
  IL-2 analog 38
cctacttcaagttctacaaagaaaacacagctacaactggagcatttactgctggatttacagatgattttgaatggaattaataattacaagaatcccaaactcaccgcgatgctcacaaagaagttttacatgcccaagaaggccacagaactgaaacatcttcagtgtctagaagaagaactcaaacctctggaggaagtgctaaatttagctcaaagcaaaaactttcacttagaccccagggacttaatcagcaatatcaacgtatttgttttcgaatttaagggatctgaaacaacattcatgtgtgaatatgctgatgagacagcaaccattgtagaatttctgaacagatggattacctttagtcaaagcatcatctcaacactgacttga

SEQ ID NO: 145 - DNA, 399 bp, Artificial Sequence
  IL-2 analog 39
cctacttcaagttctacaaagaaaacacagctacaactggagcatttactgctggatttacagatgattttgaatggaattaataattacaagaatcccaaactcaccgcgatgctcacaaagaagttttacatgcccaagaaggccacagaactgaaacatcttcagtgtctagaagaagaactcaaacctctggaggaagtgctaaatttagctcaaagcaaaaactttcacttagaccccagggacttaatcagcaatatcaacgtatttgttttcgaagtaaagggatctgaaacaacattcatgtgtgaatatgctgatgagacagcaaccattgtagaatttctgaacagatggattacctttagtcaaagcatcatctcaacactgacttga

SEQ ID NO: 146 - DNA, 399 bp, Artificial Sequence
  IL-2 analog 40
cctacttcaagttctacaaagaaaacacagctacaactggagcatttactgctggatttacagatgattttgaatggaattaataattacaagaatcccaaactcaccgcgatgctcacaaagaagttttacatgcccaagaaggccacagaactgaaacatcttcagtgtctagaagaagaactcaaacctctggaggaagtgctaaatttagctcaaagcaaaaactttcacttagaccccagggacttaatcagcaatatcaacgtatttgttttcgaaattaagggatctgaaacaacattcatgtgtgaatatgctgatgagacagcaaccattgtagaatttctgaacagatggattacctttagtcaaagcatcatctcaacactgacttga

SEQ ID NO: 147 - DNA, 399 bp, Artificial Sequence
  IL-2 analog 41
cctacttcaagttctacaaagaaaacacagctacaactggagcatttactgctggatttacagatgattttgaatggaattaataattacaagaatcccaaactcaccaggatgctcacatttaagttttacatgcccaagaaggccacagaactgaaacatcttcagtgtctagaagaagaactcaaacctctggaggaagtgctaaatttagctcaaagcaaaaactttcactttgaccccagggacgtagtcagcaatatcaacgtatttgttctggaactaaagggatctgaaacaacattcatgtgtgaatatgctgatgagacagcaaccattgtagaatttctgaacagatggattacctttagtcaaagcatcatctcaacactgacttga

SEQ ID NO: 148 - DNA, 399 bp, Artificial Sequence
  IL-2 analog 42
cctacttcaagttctacaaagaaaacacagctacaactggagcatttactgctggatttacagatgattttgaatggaattaataattacaagaatcccaaactcaccgcgatgctcacaaagaagttttacatgcccaagaaggccacagaactgaaacatcttcagtgtctagaagaagaactcaaacctctggaggaagtgctaaatttagctcaaagcaaaaactttcacttagaacccagggacttaatcagcaatatcaacgtatttgttctggaactaaagggatctgaaacaacattcatgtgtgaatatgctgatgagacagcaaccattgtagaatttctgaacagatggattacctttagtcaaagcatcatctcaacactgacttga

SEQ ID NO: 149 - DNA, 399 bp, Artificial Sequence; identical to SEQ ID NO: 143
  IL-2 analog 43

SEQ ID NO: 150 - DNA, 399 bp, Artificial Sequence
  IL-2 analog 44
cctacttcaagttctacaaagaaaacacagctacaactggagcatttactgctggatttacagatgattttgaatggaattaataattacaagaatcccaaactcaccgcgatgctcacaaagaagttttacatgcccaagaaggccacagaactgaaacatcttcagtgtctagaagaagaactcaaacctctggaggaagtgctaaatttagctcaaagcaaaaactttcacttagaccccagggtcttaatcagcaatatcaacgtatttgttctggaactaaagggatctgaaacaacattcatgtgtgaatatgctgatgagacagcaaccattgtagaatttctgaacagatggattacctttagtcaaagcatcatctcaacactgacttga

SEQ ID NO: 151 - DNA, 399 bp, Artificial Sequence
  IL-2 analog 45
cctacttcaagttctacaaagaaaacacagctacaactggagcatttactgctggatttacagatgattttgaatggaattaataattacaagaatcccaaactcaccgcgatgctcacaaagaagttttacatgcccaagaaggccacagaactgaaacatcttcagtgtctagaagaagaactcaaacctctggaggaagtgctaaatttagctcaaagcaaaaactttcacttagaccccaggttcttaatcagcaatatcaacgtatttgttctggaactaaagggatctgaaacaacattcatgtgtgaatatgctgatgagacagcaaccattgtagaatttctgaacagatggattacctttagtcaaagcatcatctcaacactgacttga

SEQ ID NO: 152 - DNA, 399 bp, Artificial Sequence
  IL-2 analog 46
cctacttcaagttctacaaagaaaacacagctacaactggagcatttactgctggttttacagatgattttgaatggaattaataattacaagaatcccaaactcaccgcgatgctcacaaagaagttttacatgcccaagaaggccacagaactgaaacatcttcagtgtctagaagaagaactcaaacctctggaggaagtgctaaatttagctcaaagcaaaaactttcacttagaccccagggacttaatcagcaatatcaacgtatttgttctggaactaaagggatctgaaacaacattcatgtgtgaatatgctgatgagacagcaaccattgtagaatttctgaacagatggattacctttagtcaaagcatcatctcaacactgacttga

SEQ ID NO: 153 - DNA, 399 bp, Artificial Sequence
  IL-2 analog 47
cctacttcaagttctacaaagaaaacacagctacaactggagcatttactgctgtttttacagatgattttgaatggaattaataattacaagaatcccaaactcaccgcgatgctcacaaagaagttttacatgcccaagaaggccacagaactgaaacatcttcagtgtctagaagaagaactcaaacctctggaggaagtgctaaatttagctcaaagcaaaaactttcacttagaccccagggacttaatcagcaatatcaacgtatttgttctggaactaaagggatctgaaacaacattcatgtgtgaatatgctgatgagacagcaaccattgtagaatttctgaacagatggattacctttagtcaaagcatcatctcaacactgacttga

SEQ ID NO: 154 - DNA, 399 bp, Artificial Sequence
  IL-2 analog 48
cctacttcaagttctacaaagaaaacacagctacaactggagcatttactgctggatttacagatgattttgaatggaattaataattacaagaatcccaaactcaccgcgatgctcacaaagaagttttacatgcccaagaaggccacagaactgaaacatcttcagtgtctagaagaagaactcaaacctctggaggaagtgctaaatttagctcaaagcaaaaactttcacttagaccccagggacttaatcagcgttatcaacgtatttgttctggaactaaagggatctgaaacaacattcatgtgtgaatatgctgatgagacagcaaccattgtagaatttctgaacagatggattacctttagtcaaagcatcatctcaacactgacttga

SEQ ID NO: 155 - DNA, 399 bp, Artificial Sequence
  IL-2 analog 49
cctacttcaagttctacaaagaaaacacagctacaactggagcatttactgctggatttacagatgattttgaatggaattaataattacaagaatcccaaactcaccgcgatgctcacaaagaagttttacatgcccaagaaggccacagaactgaaacatcttcagtgtctagaagaagaactcaaacctctggaggaagtgctaaatttagctcaaagcaaaaactttcacttagaccccagggacttaatcagctttatcaacgtatttgttctggaactaaagggatctgaaacaacattcatgtgtgaatatgctgatgagacagcaaccattgtagaatttctgaacagatggattacctttagtcaaagcatcatctcaacactgacttga

SEQ ID NO: 156 - DNA, 399 bp, Artificial Sequence
  IL-2 analog 50
cctacttcaagttctacaaagaaaacacagctacaactggagcatttactgctggatttacagatgattttgaatggaattaataattacaagaatcccaaactcaccaggatgctcacaaagaagttttacatgcccaagaaggccacagaactgaaacatcttcagtgtctagaagaagaactcaaacctctggaggaagtgctaaatttagctcaaagcaaaaactttcactttgaccccagggacgtagtcagcaatatcaacgtatttgttctggaactaaagggatctgaaacaacattcatgtgtgaatatgctgatgagacagcaaccattgtagaatttctgaacagatggattacctttagtcaaagcatcatctcaacactgacttga

SEQ ID NO: 157 - DNA, 399 bp, Artificial Sequence
  IL-2 analog 51
cctacttcaagttctacaaagaaaacacagctacaactggagcatttactgctggatttacagatgattttgaatggaattaataattacaagaatcccaaactcaccaggatgctcacatttaagttttacatgcccaagaaggccacagaactgaaacatcttcagtgtctagaacaggaactcaaacctctggaggaagtgctaaatttagctcaaagcaaaaactttcacttagaccccagggacttaatcagcaatatcaacgtatttgttctggaactaaagggatctgaaacaacattcatgtgtgaatatgctgatgagacagcaaccattgtagaatttctgaacagatggattacctttagtcaaagcatcatctcaacactgacttga

SEQ ID NO: 158 - DNA, 399 bp, Artificial Sequence
  IL-2 analog 52
cctacttcaagttctacaaagaaaacacagctacaactggagcatttactgctggatttacagatgattttgaatggaattaataattacaagaatcccaaactcaccgcgatgctcacaaagaagttttacatgcccaagaaggccacagaactgaaacatcttcagtgtctagaagaagaactcaaacctctggaggaagtgctaaatttagctcaaagcaaaaactttcactttgaccccagggacttaatcagcaatatcaacgtatttgttctggaactaaagggatctgaaacaacattcatgtgtgaatatgctgatgagacagcaaccattgtagaatttctgaacagatggattacctttagtcaaagcatcatctcaacactgacttga

SEQ ID NO: 159 - DNA, 399 bp, Artificial Sequence
  IL-2 analog 53
cctacttcaagttctacaaagaaaacacagctacaactggagcatttactgctggatttacagatgattttgaatggaattaataattacaagaatcccaaactcaccgcgatgctcacaaagaagttttacatgcccaagaaggccacagaactgaaacatcttcagtgtctagaagaagaactcaaacctctggaggaagtgctaaatttagctcaaagcaaaaactttcactttgaccccagggagttaatcagcaatatcaacgtatttgttctggaactaaagggatctgaaacaacattcatgtgtgaatatgctgatgagacagcaaccattgtagaatttctgaacagatggattacctttagtcaaagcatcatctcaacactgacttga

SEQ ID NO: 160 - DNA, 399 bp, Artificial Sequence
  IL-2 analog 54
cctacttcaagttctacaaagaaaacacagctacaactggagcatttactgctggatttacagatgattttgaatggaattaataattacaagaatcccaaactcaccgcgatgctcacaaagaagttttacatgcccaagaaggccacagaactgaaacatcttcagtgtctagaagaagaactcaaacctctggaggaagtgctaaatttagctcacagcaaaaactttcacttagaccccagggacttaatcagcaatatcaacgtatttgttctggaactaaagggatctgaaacaacattcatgtgtgaatatgctgatgagacagcaaccattgtagaatttctgaacagatggattacctttagtcaaagcatcatctcaacactgacttga

SEQ ID NO: 161 - DNA, 399 bp, Artificial Sequence
  IL-2 analog 55
cctacttcaagttctacaaagaaaacacagctacaactggagcatttactgctggatttacagatgattttgaatggaattaataattacaagaatcccaaactcaccgcgatgctcacaaagaagttttacatgcccaagaaggccacagaactgaaacatcttcagtgtctagaagaagaactcaaacctctggaggaagtgctaaatttagctcacagcaaaaactttcactttgaccccagggacttaatcagcaatatcaacgtatttgttctggaactaaagggatctgaaacaacattcatgtgtgaatatgctgatgagacagcaaccattgtagaatttctgaacagatggattacctttagtcaaagcatcatctcaacactgacttga

SEQ ID NO: 162 - DNA, 399 bp, Artificial Sequence
  IL-2 analog 56
cctacttcaagttctacaaagaaaacacagctacaactggagcatttactgctggatttacagatgattttgaatggaattaataattacaagaatcccaaactcaccgcgatgctcacaaagaagtttgccatgcccaagaaggccacagaactgaaacatcttcagtgtctagaagaagaactcaaacctctggaggaagtgctaaatttagctcacagcaaaaactttcacttagaccccagggacttaatcagcaatatcaacgtatttgttctggaactaaagggatctgaaacaacattcatgtgtgaatatgctgatgagacagcaaccattgtagaatttctgaacagatggattacctttagtcaaagcatcatctcaacactgacttga

SEQ ID NO: 163 - DNA, 399 bp, Artificial Sequence
  IL-2 analog 57
cctacttcaagttctacaaagaaaacacagctacaactggagcatttactgctggatttacagatgattttgaatggaattaataattacaagaatcccaaactcaccgcgatgctcacaaagaagtttgccatgcccaagaaggccacagaactgaaacatcttcagtgtctagaagaagaactcaaacctctggaggaagtgctaaatttagctcacagcaaaaactttcactttgaccccagggacttaatcagcaatatcaacgtatttgttctggaactaaagggatctgaaacaacattcatgtgtgaatatgctgatgagacagcaaccattgtagaatttctgaacagatggattacctttagtcaaagcatcatctcaacactgacttga

SEQ ID NO: 164 - DNA, 399 bp, Artificial Sequence
  IL-2 analog 58
cctacttcaagttctacaaagaaaacacagctacaactggagcatttactgctggatttacagatgattttgaatggaattaataattacaagaatcccaaactcaccgcgatgctcacaaagaagttttacatgcccaagaaggccacagaactgaaacatcttcagtgtctagaagaagaactcaaacctctggaggaagtgctaaatttagctcaaagcaaaaactttcactttgaccccagggacgctgccagcaatatcaacgtatttgttctggaactaaagggatctgaaacaacattcatgtgtgaatatgctgatgagacagcaaccattgtagaatttctgaacagatggattacctttagtcaaagcatcatctcaacactgacttga

SEQ ID NO: 165 - DNA, 399 bp, Artificial Sequence
  IL-2 analog 59
cctacttcaagttctacaaagaaaacacagctacaactggagcatttactgctggatttacagatgattttgaatggaattaataattacaagaatcccaaactcaccgcgatgctcacaaagaagttttacatgcccaagaaggccacagaactgaaacatcttcagtgtctagaagaagaactcaaacctctggaggaagtgctaaatttagctcaaagcaaaaactttcactttgaccccagggacgctgccagcaatatcaacgtatatgttctggaactaaagggatctgaaacaacattcatgtgtgaatatgctgatgagacagcaaccattgtagaatttctgaacagatggattacctttagtcaaagcatcatctcaacactgacttga

SEQ ID NO: 166 - DNA, 399 bp, Artificial Sequence
  IL-2 analog 60
cctacttcaagttctacaaagaaaacacagctacaactggagcatttactgctggatttacagatgattttgaatggaattaataattacaagaatcccaaactcaccgcgatgctcacaaagaagtttgccatgcccaagaaggccacagaactgaaacatcttcagtgtctagaagaagaactcaaacctctggaggaagtgctaaatttagctcaaagcaaaaactttcactatagacccagggacgctgccagcaatatcaacgtatatgttctggaactaaagggatctgaaacaacattcatgtgtgaatatgctgatgagacagcaaccattgtagaatttctgaacagatggattacctttagtcaaagcatcatctcaacactgacttga

SEQ ID NO: 167 - DNA, 399 bp, Artificial Sequence
  IL-2 analog 61
cctacttcaagttctacaaagaaaacacagctacaactggagcatttactgctggatttacagatgattttgaatggaattaataattacaagaatcccaaactcaccgcgatgctcacaaagaagttttacatgcccaagaaggccacagaactgaaacatcttcagtgtctagaagaagaactcaaacctctggaggaagtgctaaatttagctcaaagcaaaaactttcactatgaccccagggacggtgttagcaatatcaacgtatatgttctggaactaaagggatctgaaacaacattcatgtgtgaatatgctgatgagacagcaaccattgtagaatttctgaacagatggattacctttagtcaaagcatcatctcaacactgacttga

SEQ ID NO: 168 - DNA, 399 bp, Artificial Sequence
  IL-2 analog 62
cctacttcaagttctacaaagaaaacacagctacaactggagcatttactgctggatttacagatgattttgaatggaattaataattacaagaatcccaaactcaccgcgatgctcacaaagaagttttacatgcccaagaaggccacagaactgaaacatcttcagtgtctagaagaagaactcaaacctctggaggaagtgctaaatttagctcaaagcaaaaactttcactgggaacccagggacggagccagcaatatcaacgtatttgttctggaactaaagggatctgaaacaacattcatgtgtgaatatgctgatgagacagcaaccattgtagaatttctgaacagatggattacctttagtcaaagcatcatctcaacactgacttga

SEQ ID NO: 169 - DNA, 399 bp, Artificial Sequence
  IL-2 analog 63
cctacttcaagttctacaaagaaaacacagctacaactggagcatttactgctggatttacagatgattttgaatggaattaataattacaagaatcccaaactcaccgcgatgctcacaaagaagttttacatgcccaagaaggccacagaactgaaacatcttcagtgtctagaagaagaactcaaacctctggaggaagtgctaaatttagctcaaagcaaaaactttcacgacgaacccagggacacaggcagcaatatcaacgtatttgttctggaactaaagggatctgaaacaacattcatgtgtgaatatgctgatgagacagcaaccattgtagaatttctgaacagatggattacctttagtcaaagcatcatctcaacactgacttga

SEQ ID NO: 170 - DNA, 399 bp, Artificial Sequence
  IL-2 analog 64
cctacttcaagttctacaaagaaaacacagctacaactggagcatttactgctggatttacagatgattttgaatggaattaataattacaagaatcccaaactcaccgcgatgctcacaaagaagttttacatgcccaagaaggccacagaactgaaacatcttcagtgtctagaagaagaactcaaacctctggaggaagtgctaaatttagctcaaagcaaaaactttcactacaaccccagggacgtagtcagcaatatcaacgtatttgttctggaactaaagggatctgaaacaacattcatgtgtgaatatgctgatgagacagcaaccattgtagaatttctgaacagatggattacctttagtcaaagcatcatctcaacactgacttga

SEQ ID NO: 171 - DNA, 399 bp, Artificial Sequence
  IL-2 analog 65
cctacttcaagttctacaaagaaaacacagctacaactggagcatttactgctggatttacagatgattttgaatggaattaataattacaagaatcccaaactcaccgcgatgctcacaaagaagttttacatgcccaagaaggccacagaactgaaacatcttcagtgtctagaagaagaactcaaacctctggaggaagtgctaaatttagctcaaagcaaaaactttcactacgaacccagggacgtagtcagcaatatcaacgtatttgttctggaactaaagggatctgaaacaacattcatgtgtgaatatgctgatgagacagcaaccattgtagaatttctgaacagatggattacctttagtcaaagcatcatctcaacactgacttga

SEQ ID NO: 172 - DNA, 399 bp, Artificial Sequence
  IL-2 analog 66
cctacttcaagttctacaaagaaaacacagctacaactggagcatttactgctggatttacagatgattttgaatggaattaataattacaagaatcccaaactcaccgcgatgctcacaaagaagttttacatgcccaagaaggccacagaactgaaacatcttcagtgtctagaagaagaactcaaacctctggaggaagtgctaaatttagctcaaagcaaaaactttcacttcgaacccagggacttcgtcagcaatatcaacgtatttgttctggaactaaagggatctgaaacaacattcatgtgtgaatatgctgatgagacagcaaccattgtagaatttctgaacagatggattacctttagtcaaagcatcatctcaacactgacttga

SEQ ID NO: 173 - DNA, 399 bp, Artificial Sequence
  IL-2 analog 67
cctacttcaagttctacaaagaaaacacagctacaactggagcatttactgctggatttacagatgattttgaatggaattaataattacaagaatcccaaactcaccgcgatgctcacaaagaagttttacatgcccaagaaggccacagaactgaaacatcttcagtgtctagaagaagaactcaaacctctggaggaagtgctaaatttagctcaaagcaaaaactttcactatgaccccagggacttcgtcagcaatatcaacgtatgggttctggacctaaagggatctgaaacaacattcatgtgtgaatatgctgatgagacagcaaccattgtagaatttctgaacagatggattacctttagtcaaagcatcatctcaacactgacttga

SEQ ID NO: 174 - DNA, 399 bp, Artificial Sequence
  IL-2 analog 68
cctacttcaagttctacaaagaaaacacagctacaactggagcatttactgctggatttacagatgattttgaatggaattaataattacaagaatcccaaactcaccgcgatgctcacaaagaagttttacatgcccaagaaggccacagaactgaaacatcttcagtgtctagaagaagaactcaaacctctggaggaagtgctaaatttagctcaaagcaaaaactttcacttcgaacccagggacatagtcagcaatatcaacgaattcgttctggaactaaagggatctgaaacaacattcatgtgtgaatatgctgatgagacagcaaccattgtagaatttctgaacagatggattacctttagtcaaagcatcatctcaacactgacttga

SEQ ID NO: 175 - DNA, 399 bp, Artificial Sequence
  IL-2 analog 69
cctacttcaagttctacaaagaaaacacagctacaactggagcatttactgctggatttacagatgattttgaatggaattaataattacaagaatcccaaactcaccgcgatgctcacaaagaagttttacatgcccaagaaggccacagaactgaaacatcttcagtgtctagaagaagaactcaaacctctggaggaagtgctaaatttagctcaaagcaaaaactttcactacgaacccagggacttcctcagcaatatcaacgaatgggttctggacctaaagggatctgaaacaacattcatgtgtgaatatgctgatgagacagcaaccattgtagaatttctgaacagatggattacctttagtcaaagcatcatctcaacactgacttga

SEQ ID NO: 176 - DNA, 399 bp, Artificial Sequence
  IL-2 analog 70
cctacttcaagttctacaaagaaaacacagctacaactggagcatttactgctggatttacagatgattttgaatggaattaataattacaagaatcccaaactcaccgcgatgctcacaaagaagttttacatgcccaagaaggccacagaactgaaacatcttcagtgtctagaagaagaactcaaacctctggaggaagtgctaaatttagctcaaagcaaaaactttcactatgaccccagggacgtagtcagcaatatcaacgtatttgttctggaactaaagggatctgaaacaacattcatgtgtgaatatgctgatgagacagcaaccattgtagaatttctgaacagatggattacctttagtcaaagcatcatctcaacactgacttga

SEQ ID NO: 177 - DNA, 399 bp, Artificial Sequence
  IL-2 analog 71
cctacttcaagttctacaaagaaaacacagctacaactggagcatttactgctggatttacagatgattttgaatggaattaataattacaagaatcccaaactcaccgcgatgctcacaaagaagttttacatgcccaagaaggccacagaactgaaacatcttcagtgtctagaagaagaactcaaacctctggaggaagtgctaaatttagctcaaagcaaaaactttcacttcgaacccagggacgtagtcagcaatatcaacgtatttgttctggaactaaagggatctgaaacaacattcatgtgtgaatatgctgatgagacagcaaccattgtagaatttctgaacagatggattacctttagtcaaagcatcatctcaacactgacttga

SEQ ID NO: 178 - DNA, 399 bp, Artificial Sequence
  IL-2 analog 72
cctacttcaagttctacaaagaaaacacagctacaactggagcatttactgctggatttacagatgattttgaatggaattaataattacaagaatcccaaactcaccgcgatgctcacaaagaagttttacatgcccaagaaggccacagaactgaaacatcttcagtgtctagaagaagaactcaaacctctggaggaagtgctaaatttagctcaaagcaaaaactttcactttgaccccagggacgtaggcagcaatatcaacgtatttgttctggaactaaagggatctgaaacaacattcatgtgtgaatatgctgatgagacagcaaccattgtagaatttctgaacagatggattacctttagtcaaagcatcatctcaacactgacttga

SEQ ID NO: 179 - DNA, 399 bp, Artificial Sequence
  IL-2 analog 73
cctacttcaagttctacaaagaaaacacagctacaactggagcatttactgctggatttacagatgattttgaatggaattaataattacaagaatcccaaactcaccgcgatgctcacaaagaagttttacatgcccaagaaggccacagaactgaaacatcttcagtgtctagaagaagaactcaaacctctggaggaagtgctaaatttagctcaaagcaaaaactttcactttgaccccagggactgggtcagcaatatcaacgtatttgttctggaactaaagggatctgaaacaacattcatgtgtgaatatgctgatgagacagcaaccattgtagaatttctgaacagatggattacctttagtcaaagcatcatctcaacactgacttga

SEQ ID NO: 180 - DNA, 399 bp, Artificial Sequence
  IL-2 analog 74
cctacttcaagttctacaaagaaaacacagctacaactggagcatttactgctggatttacagatgattttgaatggaattaataattacaagaatcccaaactcaccgatatgctcacaaagaagttttacatgcccaagaaggccacagaactgaaacatcttcagtgtctagaagaagaactcaaacctctggaggaagtgctaaatttagctcaaagcaaaaactttcactatgaccccagggacgtagtcagcaatatcaacgtatttgttctggaactaaagggatctgaaacaacattcatgtgtgaatatgctgatgagacagcaaccattgtagaatttctgaacagatggattacctttagtcaaagcatcatctcaacactgacttga

SEQ ID NO: 181 - DNA, 399 bp, Artificial Sequence
  IL-2 analog 75
cctacttcaagttctacaaagaaaacacagctacaactggagcatttactgctggatttacagatgattttgaatggaattaataattacaagaatcccaaactcaccgcgatgctcacaaagaagtttgccatgcccaagaaggccacagaactgaaacatcttcagtgtctagaagaagaactcaaacctctggaggaagtgctaaatttagctcaaagcaaaaactttcacttcgaacccagggacgtagtcagcaatatcaacgtatttgttctggaactaaagggatctgaaacaacattcatgtgtgaatatgctgatgagacagcaaccattgtagaatttctgaacagatggattacctttagtcaaagcatcatctcaacactgacttga

SEQ ID NO: 182 - DNA, 399 bp, Artificial Sequence
  IL-2 analog 76
cctacttcaagttctacaaagaaaacacagctacaactggagcatttactgctggatttacagatgattttgaatggaattaataattacaagaatcccaaactcaccgcgatgctcacaaagcagttttacatgcccaagaaggccacagaactgaaacatcttcagtgtctagaacgggaactcaaacctctggaggaagtgctaaatttagctcaaagcaaaaactttcactttgaccccagggacgtaggcagcaatatcaacgtatttgttctggaactaaagggatctgaaacaacattcatgtgtgaatatgctgatgagacagcaaccattgtagaatttctgaacagatggattacctttagtcaaagcatcatctcaacactgacttga

SEQ ID NO: 183 - DNA, 399 bp, Artificial Sequence
  IL-2 analog 77
cctacttcaagttctacaaagaaaacacagctacaactggagcatttactgctggatttacagatgattttgaatggaattaataattacaagaatcccaaactcaccgcgatgctcacaaaggagttttacatgcccaagaaggccacagaactgaaacatcttcagtgtctagaacgggaactcaaacctctggaggaagtgctaaatttagctcaaagcaaaaactttcactttgaccccagggactgggtcagcaatatcaacgtatttgttctggaactaaagggatctgaaacaacattcatgtgtgaatatgctgatgagacagcaaccattgtagaatttctgaacagatggattacctttagtcaaagcatcatctcaacactgacttga

SEQ ID NO: 184 - DNA, 399 bp, Artificial Sequence
  IL-2 analog 78
cctacttcaagttctacaaagaaaacacagctacaactggagcatttactgctggatttacagatgattttgaatggaattaataattacaagaatcccgaactcaccgcgatgctcacaaagaagttttacatgcccaagaaggccacagaactgaaacatcttcagtgtctagaagaagaactcaaacctctggaggaagtgctaaatttagctcaaagcaaaaactttcacttcgaacccagggacgtagtcagcaatatcaacgtatttgttctggaactaaagggatctgaaacaacattcatgtgtgaatatgctgatgagacagcaaccattgtagaatttctgaacagatggattacctttagtcaaagcatcatctcaacactgacttga

SEQ ID NO: 185 - DNA, 399 bp, Artificial Sequence
  IL-2 analog 79
cctacttcaagttctacaaagaaaacacagctacaactggagcatttactgctggatttacagatgattttgaatggaattaataattacaagaatcccgaactcaccgcgatgctcacaaagaagttttacatgcccaagaaggccacagaactgaaacatcttcagtgtctagaagaagaactcaaacctctggaggaagtgctaaatttagctcacagcaaaaactttcacttcgaacccagggacgtagtcagcaatatcaacgtatttgttctggaactaaagggatctgaaacaacattcatgtgtgaatatgctgatgagacagcaaccattgtagaatttctgaacagatggattacctttagtcaaagcatcatctcaacactgacttga

SEQ ID NO: 186 - DNA, 399 bp, Artificial Sequence
  IL-2 analog 80
cctacttcaagttctacaaagaaaacacagctacaactggagcatttactgctggatttacagatgattttgaatggaattaataattacaagaatcccgaactcaccgcgatgctcacaaagaagttttacatgcccaagaaggccacagaactgaaacatcttcagtgtctagaagaagaactcaaacctctggaggaagtgctaaatttagctcacagcaaaaactttcacttcgaaggcagggacgtagtcagcaatatcaacgtatttgttctggaactaaagggatctgaaacaacattcatgtgtgaatatgctgatgagacagcaaccattgtagaatttctgaacagatggattacctttagtcaaagcatcatctcaacactgacttga

SEQ ID NO: 187 - DNA, 399 bp, Artificial Sequence
  IL-2 analog 81
cctacttcaagttctacaaagaaaacacagctacaactggagcatttactgctggatttacagatgattttgaatggaattaataattacaagaatcccgaactcaccgcgatgctcacaaagaagttttacatgcccaagaaggccacagaactgaaacatcttcagtgtctagaagaagaactcaaacctctggaggaagtgctaaatttagctcacagcaaaaactttcacttcgaagtcagggacgtagtcagcaatatcaacgtatttgttctggaactaaagggatctgaaacaacattcatgtgtgaatatgctgatgagacagcaaccattgtagaatttctgaacagatggattacctttagtcaaagcatcatctcaacactgacttga

SEQ ID NO: 188 - DNA, 399 bp, Artificial Sequence
  IL-2 analog 82
cctacttcaagttctacaaagaaaacacagctacaactggagcatttacgtctggatttagaaatgattttgaatggaattaataattacaagaatcccaaactcaccaggatgctcacatttaagttttacatgcccaagaaggccacagaactgaaacatcttcagtgtctagaagaagaactcaaacctctggaggaagtgctaaatttagctcaaagcaaaaactttcactttgaccccagggacgaagtgagcaatatcaacgtatttgttctggaactaaagggatctgaaacaacattcatgtgtgaatatgctgatgagacagcaaccattgtagaatttctgaacagatggattacctttagtcaaagcatcatctcaacactgacttga

SEQ ID NO: 189 - DNA, 399 bp, Artificial Sequence
  IL-2 analog 83
cctacttcaagttctacaaagaaaacacagctacaactggagcatttacgtcgtgatttagaaatgattttgaatggaattaataattacaagaatcccaaactcaccaggatgctcacatttaagttttacatgcccaagaaggccacagaactgaaacatcttcagtgtctagaagaagaactcaaacctctggaggaagtgctaaatttagctcaaagcaaaaactttcactttgaccccagggacgaagtgagcaatatcaacgtatttgttctggaactaaagggatctgaaacaacattcatgtgtgaatatgctgatgagacagcaaccattgtagaatttctgaacagatggattacctttagtcaaagcatcatctcaacactgacttga

SEQ ID NO: 190 - DNA, 399 bp, Artificial Sequence
  IL-2 analog 84
cctacttcaagttctacaaagaaaacacagctacaactggagcatttacgtctggatttagaaatgattttgaatggaattaataattacaagaatcccaaactcaccaggatgctcacatttaagttttacatgcccaagaaggccacagaactgaaacatcttcagtgtctagaagaagaactcaaacctctggaggaagtgctaaatttagctcaaagcaaaaactttcacgtggatcccagggacgaagtgagcaatatcaacgtatttgttctggaactaaagggatctgaaacaacattcatgtgtgaatatgctgatgagacagcaaccattgtagaatttctgaacagatggattacctttagtcaaagcatcatctcaacactgacttga

SEQ ID NO: 191 - DNA, 399 bp, Artificial Sequence
  IL-2 analog 85
cctacttcaagttctacaaagaaaacacagctacaactggagcatttactgctggatttacagatgattttgaatggaattaataattacaagaatcccaaactcaccaggatgctcacatttaagttttacatgcccaagaaggccacagaactgaaacatcttcagtgtctagaagaagaactcaaacctctggaggaagtgctaaatttagctcaaagcaaaaactttcacttcgaacccagggacgtagtcagcaatatcaacgtatttgttctggaactaaagggatctgaaacaacattcatgtgtgaatatgctgatgagacagcaaccattgtagaatttctgaacagatggattacctttagtcaaagcatcatctcaacactgacttga

SEQ ID NO: 192 - DNA, 399 bp, Artificial Sequence
  IL-2 analog 86
cctacttcaagttctacaaagaaaacacagctacaactggagcatttacgtctggatttagaaatgattttgaatggaattaataattacaagaatcccaaactcaccaggatgctcacatttaagttttacatgcccaagaaggccacagaactgaaacatcttcagtgtctagaagaagaactcaaacctctggaggaagtgctaaatttagctcaaagcaaaaactttcacttcgaacccagggacgtagtcagcaatatcaacgtatttgttctggaactaaagggatctgaaacaacattcatgtgtgaatatgctgatgagacagcaaccattgtagaatttctgaacagatggattacctttagtcaaagcatcatctcaacactgacttga

SEQ ID NO: 193 - DNA, 399 bp, Artificial Sequence
  IL-2 analog 87
cctacttcaagttctacaaagaaaacacagctacaactggagcatttacgtcgtgatttagaaatgattttgaatggaattaataattacaagaatcccaaactcaccaggatgctcacatttaagttttacatgcccaagaaggccacagaactgaaacatcttcagtgtctagaagaagaactcaaacctctggaggaagtgctaaatttagctcaaagcaaaaactttcacttcgaacccagggacgtagtcagcaatatcaacgtatttgttctggaactaaagggatctgaaacaacattcatgtgtgaatatgctgatgagacagcaaccattgtagaatttctgaacagatggattacctttagtcaaagcatcatctcaacactgacttga

SEQ ID NO: 194 - DNA, 399 bp, Artificial Sequence
  IL-2 analog 88
cctacttcaagttctacaaagaaaacacagctacaactggagcatttactgctggatttacagatgattttgaatggaattaataattacaagaatcccaaactcaccaggatgctcacatttaagttttacatgcccaagaaggccacagaactgaaacatcttcagtgtctagaagacgaactcaaacctctggaggaagtgctaaatttagctcaaagcaaaaactttcacttcgaacccagggacgtagtcagcaatatcaacgtatttgttctggaactaaagggatctgaaacaacattcatgtgtgaatatgctgatgagacagcaaccattgtagaatttctgaacagatggattacctttagtcaaagcatcatctcaacactgacttga

SEQ ID NO: 195 - DNA, 399 bp, Artificial Sequence
  IL-2 analog 89
cctacttcaagttctacaaagaaaacacagctacaactggagcatttactgctggatttacagatgattttgaatggaattaataattacaagaatcccaaactcaccgcgatgctcacatttaagttttacatgcccaagaaggccacagaactgaaacatcttcagtgtctagaagaagaactcaaacctctggagcaggtgctaaatttagctcaaagcaaaaactttcacttcgaacccagggacgtagtcagcaatatcaacgtatttgttctggaactaaagggatctgaaacaacattcatgtgtgaatatgctgatgagacagcaaccattgtagaatttctgaacagatggattacctttagtcaaagcatcatctcaacactgacttga

SEQ ID NO: 196 - DNA, 399 bp, Artificial Sequence
  IL-2 analog 90
cctacttcaagttctacaaagaaaacacagctacaactggagcatttactgctggatttacagatgattttgaatggaattaataattacaagaatcccaaactcaccaggatgctcacatggaagttttacatgcccaagaaggccacagaactgaaacatcttcagtgtctagaagaagaactcaaacctctggaggaagtgctaaatttagctcaaagcaaaaactttcacttcgaacccagggacgtagtcagcaatatcaacgtatttgttctggaactaaagggatctgaaacaacattcatgtgtgaatatgctgatgagacagcaaccattgtagaatttctgaacagatggattacctttagtcaaagcatcatctcaacactgacttga

SEQ ID NO: 197 - DNA, 399 bp, Artificial Sequence
  IL-2 analog 91
cctacttcaagttctacaaagaaaacacagctacaactggagcatttactgctggatttacagatgattttgaatggaattaataattacaagaatcccaaactcaccaggatgctcacatttaagttttacatgcccaagaaggccacagaactgaaacatcttcagtgtctagaacaagaactcaaacctctggaggaagtgctaaatttagctcaaagcaaaaactttcacttcgaacccagggacgtagtcagcaatatcaacgtatttgttctggaactaaagggatctgaaacaacattcatgtgtgaatatgctgatgagacagcaaccattgtagaatttctgaacagatggattacctttagtcaaagcatcatctcaacactgacttga

SEQ ID NO: 198 - DNA, 399 bp, Artificial Sequence
  IL-2 analog 92
cctacttcaagttctacaaagaaaacacagctacaactggagcatttactgctggatttacagatgattttgaatggaattaataattacaagaatcccaaactcaccaggatgctcacatttaagttttacatgcccaagaaggccacagaactgaaacatcttcagtgtctagaagaagaactcaaacctctggaggaagtgctaaatttagctcaaagcaaaaactttcacttcgaacccagggacgtagtcagcaatatcaacacatttgttctggaactaaagggatctgaaacaacattcatgtgtgaatatgctgatgagacagcaaccattgtagaatttctgaacagatggattacctttagtcaaagcatcatctcaacactgacttga

SEQ ID NO: 199 - DNA, 399 bp, Artificial Sequence
  IL-2 analog 93
cctacttcaagttctacaaagaaaacacagctacaactggagcatttactgctggatttacagatgattttgaatggaattaataattacaagaatcccaaactcaccaggatgctcacatttaagttttacatgcccaagaaggccacagaactgaaacatcttcagtgtctagaagaagaactcaaacctctggaggaagtgctaaatttagctcaaagcaaaaactttcacttcgaacccagggaggtagtcagcaatatcaacacatttgttctggaactaaagggatctgaaacaacattcatgtgtgaatatgctgatgagacagcaaccattgtagaatttctgaacagatggattacctttagtcaaagcatcatctcaacactgacttga

SEQ ID NO: 200 - DNA, 399 bp, Artificial Sequence
  IL-2 analog 94
cctacttcaagttctacaaagaaaacacagctacaactggagcatttactgctggatttacagatgattttgaatggaattaataattacaagaatcccaaactcaccaggatgctcacatttaagttttacatgcccaagaaggccacagaactgaaacatcttcagtgtctagaagaagaactcaaacctctggaggaagtgctaaatttagctcaaagcaaaaactttcacttcgaacccagggacgtagtcagcaatatcaacgtatttgttttcgaattcaagggatctgaaacaacattcatgtgtgaatatgctgatgagacagcaaccattgtagaatttctgaacagatggattacctttagtcaaagcatcatctcaacactgacttga

SEQ ID NO: 201 - DNA, 399 bp, Artificial Sequence
  IL-2 analog 95
cctacttcaagttctacaaagaaaacacagctacaactggagcatttactgctggatttacagatgattttgaatggaattaataattacaagaatcccaaactcaccaggatgctcacatttaagttttacatgcccaagaaggccacagaactgaaacatcttcagtgtctagaagaagaactcaaacctctggaggaagggctaaatttagctcaaagcaaaaactttcacttcgaacccagggacgtagtcagcaatatcaacgtatttgttctggaactaaagggatctgaaacaacattcatgtgtgaatatgctgatgagacagcaaccattgtagaatttctgaacagatggattacctttagtcaaagcatcatctcaacactgacttga

SEQ ID NO: 202 - DNA, 399 bp, Artificial Sequence
  IL-2 analog 96
cctacttcaagttctacaaagaaaacacagctacaactggagcatttactgctggatttacagatgattttgaatggaattaataattacaagaatcccaaactcaccaggatgctcacatttaagttttacatgcccaagaaggccacagaactgaaacatcttcagtgtctagaagaagaactcaaacctctggaggaagggctaaatttagctgcaagcaaaaactttcacttcgaacccagggacgtagtcagcaatatcaacgtatttgttctggaactaaagggatctgaaacaacattcatgtgtgaatatgctgatgagacagcaaccattgtagaatttctgaacagatggattacctttagtcaaagcatcatctcaacactgacttga

SEQ ID NO: 203 - DNA, 399 bp, Artificial Sequence
  IL-2 analog 97
cctacttcaagttctacaaagaaaacacagctacaactggagcatttactgctggatttacagatgattttgaatggaattaataattacaagaatcccaaactcaccgcgatgctcacatttaagttttacatgcccaagaaggccacagaactgaaacatcttcagtgtctagaagaagaactcaaacctctggaggaagtgctaaatttagctcaaagcaaaaactttcactttgaccccagggacttaatcagcaatatcaacgtatttgttctggaactaaagggatctgaaacaacattcatgtgtgaatatgctgatgagacagcaaccattgtagaatttctgaacagatggattacctttagtcaaagcatcatctcaacactgacttga

SEQ ID NO: 204 - DNA, 399 bp, Artificial Sequence
  IL-2 analog 98
cctacttcaagttctacaaagaaaacacagctacaactggagcatttactgctggatttacagatgattttgaatggaattaataattacaagaatcccaaactcaccgcgatgctcacatttaagttttacatgcccaagaaggccacagaactgaaacatcttcagtgtctagaagaagaactcaaacctctggaggaagtgctaaatttagctcaaagcaaaaactttcactttgagcccagggacgtaatcagcaatatcaacgtatttgttctggaactaaagggatctgaaacaacattcatgtgtgaatatgctgatgagacagcaaccattgtagaatttctgaacagatggattacctttagtcaaagcatcatctcaacactgacttga

SEQ ID NO: 205 - DNA, 399 bp, Artificial Sequence
  IL-2 analog 99
cctacttcaagttctacaaagaaaacacagctacaactggagcatttactgctggatttacagatgattttgaatggaattaataattacaagaatcccaaactcaccgcgatgctcacatttaagttttacatgcccaagaaggccacagaactgaaacatcttcagtgtctagaagaagaactcaaacctctggaggaagtgctaaatttagctcaaagcaaaaactttcactttgagcccagggacttagtcagcaatatcaacgtatttgttctggaactaaagggatctgaaacaacattcatgtgtgaatatgctgatgagacagcaaccattgtagaatttctgaacagatggattacctttagtcaaagcatcatctcaacactgacttga

SEQ ID NO: 206 - DNA, 399 bp, Artificial Sequence
  IL-2 analog 100
cctacttcaagttctacaaagaaaacacagctacaactggagcatttactgctggatttacagatgattttgaatggaattaataattacaagaatcccaaactcaccaggatgctcacatttaagttttacatgcccaagaaggccacagaactgaaacatcttcagtgtctagaagaagaactcaaacctctggaggaagtgctaaatttagctcaaagcaaaaactttcacttcgaacccagggactacgtcagcaatatcaacgtatttgttctggaactaaagggatctgaaacaacattcatgtgtgaatatgctgatgagacagcaaccattgtagaatttctgaacagatggattacctttagtcaaagcatcatctcaacactgacttga

SEQ ID NO: 207 - DNA, 399 bp, Artificial Sequence
  IL-2 analog 101
cctacttcaagttctacaaagaaaacacagctacaactggagcatttactgctggatttacagatgattttgaatggaattaataattacaagaatcccaaactcaccaggatgctcacatttaagttttacatgcccaagaaggccacagaactgaaacatcttcagtgtctagaagaagaactcaaacctctggaggaagtgctaaatttagctcaaagcaaaaactttcacttcgaacccagggacctggccagcaatatcaacgtatttgttctggaactaaagggatctgaaacaacattcatgtgtgaatatgctgatgagacagcaaccattgtagaatttctgaacagatggattacctttagtcaaagcatcatctcaacactgacttga

SEQ ID NO: 208 - DNA, 399 bp, Artificial Sequence
  IL-2 analog 102
cctacttcaagttctacaaagaaaacacagctacaactggagcatttactgctggatttacagatgattttgaatggaattaataattacaagaatcccaaactcaccaggatgctcacatttaagttttacatgcccaagaaggccacagaactgaaacatcttcagtgtctagaagaagaactcaaacctctggaggaagtgctaaatttagctcaaagcaaaaactttcacttcgaacccagggacgtagtcagcaatatcaacgtaattgttctggaactaaagggatctgaaacaacattcatgtgtgaatatgctgatgagacagcaaccattgtagaatttctgaacagatggattacctttagtcaaagcatcatctcaacactgacttga

SEQ ID NO: 209 - DNA, 399 bp, Artificial Sequence
  IL-2 analog 103
cctacttcaagttctacaaagaaaacacagctacaactggagcatttacgtctggatttagaaatgattttgaatggaattaataattacaagaatcccaaactcaccgcgatgctcacatttaagttttacatgcccaagaaggccacagaactgaaacatcttcagtgtctagaagaagaactcaaacctctggaggaagtgctaaatttagctcaaagcaaaaactttcacttcgaacccagggacgtagtcagcaatatcaacgtatttgttctggaactaaagggatctgaaacaacattcatgtgtgaatatgctgatgagacagcaaccattgtagaatttctgaacagatggattacctttagtcaaagcatcatctcaacactgacttga

SEQ ID NO: 210 - DNA, 399 bp, Artificial Sequence
  IL-2 analog 104
cctacttcaagttctacaaagaaaacacagctacaactggagcatttacgtctggatttagaaatgattttgaatggaattaataattacaagaatcccaaactcaccaggatgctcacatttaagttttacatgcccaagaaggccacagaactgaaacatcttcagtgtctagaagacgaactcaaacctctggaggaagtgctaaatttagctcaaagcaaaaactttcacttcgaacccagggacgtagtcagcaatatcaacgtatttgttctggaactaaagggatctgaaacaacattcatgtgtgaatatgctgatgagacagcaaccattgtagaatttctgaacagatggattacctttagtcaaagcatcatctcaacactgacttga

SEQ ID NO: 211 - DNA, 399 bp, Artificial Sequence
  IL-2 analog 105
cctacttcaagttctacaaagaaaacacagctacaactggagcatttacgtctggatttagaaatgattttgaatggaattaataattacaagaatcccaaactcaccaggatgctcacatttaagttttacatgcccaagaaggccacagaactgaaacatcttcagtgtctagaagaagaactcaaacctctggaggacgtgctaaatttagctcaaagcaaaaactttcacttcgaacccagggacgtagtcagcaatatcaacgtatttgttctggaactaaagggatctgaaacaacattcatgtgtgaatatgctgatgagacagcaaccattgtagaatttctgaacagatggattacctttagtcaaagcatcatctcaacactgacttga

SEQ ID NO: 212 - protein, 133 aa, Artificial Sequence
  General Formula 1
  MISC_FEATURE (1): Xaa is a deletion
  MISC_FEATURE (18): Xaa is leucine (L) or arginine (R)
  MISC_FEATURE (19): Xaa is leucine (L) or tyrosine (Y)
  MISC_FEATURE (22): Xaa is glutamic acid (E) or glutamine (Q)
  MISC_FEATURE (38): Xaa is alanine (A), aspartic acid (D), or arginine (R)
  MISC_FEATURE (42): Xaa is alanine (A), phenylalanine (F), lysine (K), or tryptophan (W)
  MISC_FEATURE (43): Xaa is glutamic acid (E), lysine (K), or glutamine (Q)
  MISC_FEATURE (45): Xaa is alanine (A) or tyrosine (Y)
  MISC_FEATURE (61): Xaa is aspartic acid (D), glutamic acid (E), glutamine (Q), or arginine (R)
  MISC_FEATURE (68): Xaa is aspartic acid (D) or glutamic acid (E)
  MISC_FEATURE (74): Xaa is histidine (H) or glutamine (Q)
  MISC_FEATURE (80): Xaa is phenylalanine (F), leucine (L), valine (V), or tyrosine (Y)
  MISC_FEATURE (81): Xaa is aspartic acid (D), glutamic acid (E), or arginine (R)
  MISC_FEATURE (84): Xaa is aspartic acid (D) or glutamic acid (E)
  MISC_FEATURE (85): Xaa is alanine (A), glutamic acid (E), glycine (G), leucine (L), valine (V), tryptophan (W), or tyrosine (Y)
  MISC_FEATURE (86): Xaa is alanine (A), glycine (G), isoleucine (I), or valine (V)
  MISC_FEATURE (91): Xaa is threonine (T) or valine (V)
  MISC_FEATURE (92): Xaa is phenylalanine (F), isoleucine (I), or tyrosine (Y)
  MISC_FEATURE (94): Xaa is phenylalanine (F) or leucine (L)
  MISC_FEATURE (96): Xaa is phenylalanine (F) or leucine (L)
XPTSSSTKKTQLQLEHLXXDLXMILNGINNYKNPKLTXMLTXXFXMPKKATELKHLQCLEXELKPLEXVLNLAXSKNFHXXPRXXXSNINXXVXEXKGSETTFMCEYADETATIVEFLNRWITFSQSIISTLT

SEQ ID NO: 213 - protein, 133 aa, Artificial Sequence
  General Formula 2
  MISC_FEATURE (1): Xaa is a deletion
  MISC_FEATURE (18): Xaa is leucine (L) or arginine (R)
  MISC_FEATURE (22): Xaa is glutamic acid (E) or glutamine (Q)
  MISC_FEATURE (38): Xaa is alanine (A) or arginine (R)
  MISC_FEATURE (42): Xaa is phenylalanine (F) or lysine (K)
  MISC_FEATURE (61): Xaa is aspartic acid (D) or glutamic acid (E)
  MISC_FEATURE (68): Xaa is aspartic acid (D) or glutamic acid (E)
  MISC_FEATURE (81): Xaais aspartic acid (D) or glutamic acid (E)
  MISC_FEATURE (85): Xaa is leucine (L) or valine (V)
  MISC_FEATURE (86): Xaa is isoleucine (I) or valine (V)
XPTSSSTKKTQLQLEHLXLDLXMILNGINNYKNPKLTXMLTXKFYMPKKATELKHLQCLEXELKPLEXVLNLAQSKNFHFXPRDXXSNINVFVLELKGSETTFMCEYADETATIVEFLNRWITFSQSIISTLT

SEQ ID NO: 214 - DNA, 33 bp, Artificial Sequence
  primer #1 (IL2_L12F_F)
caaagaaaacacagtttcaactggagcatttac

SEQ ID NO: 215 - DNA, 33 bp, Artificial Sequence
  primer #2 (IL2_L12F_R)
gtaaatgctccagttgaaactgtgttttctttg

SEQ ID NO: 216 - DNA, 33 bp, Artificial Sequence
  primer #3 (IL2_L12V_F)
caaagaaaacacaggtacaactggagcatttac

SEQ ID NO: 217 - DNA, 33 bp, Artificial Sequence
  primer #4 (IL2_L12V_R)
gtaaatgctccagttgtacctgtgttttctttg

SEQ ID NO: 218 - DNA, 39 bp, Artificial Sequence
  primer #5 (IL2_L18R_L19R_Q22E_F)
ctggagcatttacgtcgtgatttagaaatgattttgaat

SEQ ID NO: 219 - DNA, 39 bp, Artificial Sequence
  primer #6 (IL2_L18R_L19R_Q22E_R)
attcaaaatcatttctaaatcacgacgtaaatgctccag

SEQ ID NO: 220 - DNA, 39 bp, Artificial Sequence
  primer #7 (IL2_L18R_Q22E_F)
ctggagcatttacgtctggatttagaaatgattttgaat

SEQ ID NO: 221 - DNA, 39 bp, Artificial Sequence
  primer #8 (IL2_L18R_Q22E_R)
attcaaaatcatttctaaatccagacgtaaatgctccag

SEQ ID NO: 222 - DNA, 33 bp, Artificial Sequence
  primer #9 (IL2_L19F_F)
gagcatttactgttcgatttacagatgattttg

SEQ ID NO: 223 - DNA, 33 bp, Artificial Sequence
  primer #10 (IL2_L19F_R)
caaaatcatctgtaaatcgaacagtaaatgctc

SEQ ID NO: 224 - DNA, 33 bp, Artificial Sequence
  primer #11 (IL2_L19V_F)
gagcatttactggtggatttacagatgattttg

SEQ ID NO: 225 - DNA, 33 bp, Artificial Sequence
  primer #12 (IL2_L19V_R)
caaaatcatctgtaaatccaccagtaaatgctc

SEQ ID NO: 226 - DNA, 33 bp, Artificial Sequence
  primer #13 (IL2_L19Y_F)
caactggagcatttactgtacgatttacagatg

SEQ ID NO: 227 - DNA, 33 bp, Artificial Sequence
  primer #14 (IL2_L19Y_R)
catctgtaaatcgtacagtaaatgctccagttg

SEQ ID NO: 228 - DNA, 34 bp, Artificial Sequence
  primer #15 (IL2_D20F_F)
ggagcatttactgctgtttttacagatgattttg

SEQ ID NO: 229 - DNA, 34 bp, Artificial Sequence
  primer #16 (IL2_D20F_R)
caaaatcatctgtaaaaacagcagtaaatgctcc

SEQ ID NO: 230 - DNA, 33 bp, Artificial Sequence
  primer #17 (IL2_D20V_F)
gagcatttactgctggttttacagatgattttg

SEQ ID NO: 231 - DNA, 33 bp, Artificial Sequence
  primer #18 (IL2_D20V_R)
caaaatcatctgtaaaaccagcagtaaatgctc

SEQ ID NO: 232 - DNA, 33 bp, Artificial Sequence
  primer #19 (IL2_K32C_F)
ggaattaataattactgtaatcccaaactcacc

SEQ ID NO: 233 - DNA, 33 bp, Artificial Sequence
  primer #20 (IL2_K32C_R)
ggtgagtttgggattacagtaattattaattcc

SEQ ID NO: 234 - DNA, 33 bp, Artificial Sequence
  primer #21 (IL2_K35C_F)
aattacaagaatccctgtctcaccaggatgctc

SEQ ID NO: 235 - DNA, 33 bp, Artificial Sequence
  primer #22 (IL2_K35C_R)
gagcatcctggtgagacagggattcttgtaatt

SEQ ID NO: 236 - DNA, 33 bp, Artificial Sequence
  primer #23 (IL2_K35E_F)
taattacaagaatcccgaactcaccgcgatgct

SEQ ID NO: 237 - DNA, 33 bp, Artificial Sequence
  primer #24 (IL2_K35E_R)
agcatcgcggtgagttcgggattcttgtaatta

SEQ ID NO: 238 - DNA, 25 bp, Artificial Sequence
  primer #25 (IL2_R38A_F)
ccaaactcaccgcgatgctcacatt

SEQ ID NO: 239 - DNA, 25 bp, Artificial Sequence
  primer #26 (IL2_R38A_R)
aatgtgagcatcgcggtgagtttgg

SEQ ID NO: 240 - DNA, 33 bp, Artificial Sequence
  primer #27 (IL2_R38A_F42F_F)
caccgcgatgctcacatttaagttttacatgcc

SEQ ID NO: 241 - DNA, 33 bp, Artificial Sequence
  primer #28 (IL2_R38A_F42F_R)
ggcatgtaaaacttaaatgtgagcatcgcggtg

SEQ ID NO: 242 - DNA, 25 bp, Artificial Sequence
  primer #29 (IL2_A38R_F)
ccaaactcaccaggatgctcacatt

SEQ ID NO: 243 - DNA, 25 bp, Artificial Sequence
  primer #30 (IL2_A38R_R)
aatgtgagcatcctggtgagtttgg

SEQ ID NO: 244 - DNA, 30 bp, Artificial Sequence
  primer #31 (IL2_R38D_F)
aagaatcccaaactcaccgatatgctcaca

SEQ ID NO: 245 - DNA, 30 bp, Artificial Sequence
  primer #32 (IL2_R38D_R)
tgtgagcatatcggtgagtttgggattctt

SEQ ID NO: 246 - DNA, 30 bp, Artificial Sequence
  primer #33 (IL2_F42A_F)
ccaggatgctcacagctaagttttacatgc

SEQ ID NO: 247 - DNA, 30 bp, Artificial Sequence
  primer #34 (IL2_F42A_R)
gcatgtaaaacttagctgtgagcatcctgg

SEQ ID NO: 248 - DNA, 30 bp, Artificial Sequence
  primer #35 (IL2_F42K_F)
ccaggatgctcacaaagaagttttacatgc

SEQ ID NO: 249 - DNA, 30 bp, Artificial Sequence
  primer #36 (IL2_F42K_R)
gcatgtaaaacttctttgtgagcatcctgg

SEQ ID NO: 250 - DNA, 30 bp, Artificial Sequence
  primer #37 (IL2_F42K_K43E_F)
atgctcacaaaggagttttacatgcccaag

SEQ ID NO: 251 - DNA, 30 bp, Artificial Sequence
  primer #38 (IL2_F42K_K43E_R)
cttgggcatgtaaaactcctttgtgagcat

SEQ ID NO: 252 - DNA, 30 bp, Artificial Sequence
  primer #39 (IL2_F42K_K43Q_F)
atgctcacaaagcagttttacatgcccaag

SEQ ID NO: 253 - DNA, 30 bp, Artificial Sequence
  primer #40 (IL2_F42K_K43Q_R)
cttgggcatgtaaaactgctttgtgagcat

SEQ ID NO: 254 - DNA, 30 bp, Artificial Sequence
  primer #41 (IL2_K42F_F)
ccaggatgctcacatttaagttttacatgc

SEQ ID NO: 255 - DNA, 30 bp, Artificial Sequence
  primer #42 (IL2_K42F_R)
gcatgtaaaacttaaatgtgagcatcctgg

SEQ ID NO: 256 - DNA, 39 bp, Artificial Sequence
  primer #43 (IL2_K42F_F_long)
ctcaccaggatgctcacatttaagttttacatgcccaag

SEQ ID NO: 257 - DNA, 39 bp, Artificial Sequence
  primer #44 (IL2_K42F_R_long)
cttgggcatgtaaaacttaaatgtgagcatcctggtgag

SEQ ID NO: 258 - DNA, 33 bp, Artificial Sequence
  primer #45 (IL2_F42W_F)
accaggatgctcacatggaagttttacatgccc

SEQ ID NO: 259 - DNA, 33 bp, Artificial Sequence
  primer #46 (IL2_F42W_R)
gggcatgtaaaacttccatgtgagcatcctggt

SEQ ID NO: 260 - DNA, 33 bp, Artificial Sequence
  primer #47 (IL2_K43C_F)
aggatgctcacattttgtttttacatgcccaag

SEQ ID NO: 261 - DNA, 33 bp, Artificial Sequence
  primer #48 (IL2_K43C_R)
cttgggcatgtaaaaacaaaatgtgagcatcct

SEQ ID NO: 262 - DNA, 19 bp, Artificial Sequence
  primer #49 (IL2_Y45A_F)
gaagtttgccatgcccaag

SEQ ID NO: 263 - DNA, 19 bp, Artificial Sequence
  primer #50 (IL2_Y45A_R)
cttgggcatggcaaacttc

SEQ ID NO: 264 - DNA, 34 bp, Artificial Sequence
  primer #51 (IL2_Y45A_F_long)
gctcacaaagaagtttgccatgcccaagaaggcc

SEQ ID NO: 265 - DNA, 34 bp, Artificial Sequence
  primer #52 (IL2_Y45A_R_long)
ggccttcttgggcatggcaaacttctttgtgagc

SEQ ID NO: 266 - DNA, 33 bp, Artificial Sequence
  primer #53 (IL2_K48C_F)
aagttttacatgccctgtaaggccacagaactg

SEQ ID NO: 267 - DNA, 33 bp, Artificial Sequence
  primer #54 (IL2_K48C_R)
cagttctgtggccttacagggcatgtaaaactt

SEQ ID NO: 268 - DNA, 33 bp, Artificial Sequence
  primer #55 (IL2_K49C_F)
ttttacatgcccaagtgtgccacagaactgaaa

SEQ ID NO: 269 - DNA, 33 bp, Artificial Sequence
  primer #56 (IL2_K49C_R)
tttcagttctgtggcacacttgggcatgtaaaa

SEQ ID NO: 270 - DNA, 33 bp, Artificial Sequence
  primer #57 (IL2_E61D_F)
cttcagtgtctagaagacgaactcaaacctctg

SEQ ID NO: 271 - DNA, 33 bp, Artificial Sequence
  primer #58 (IL2_E61D_R)
cagaggtttgagttcgtcttctagacactgaag

SEQ ID NO: 272 - DNA, 33 bp, Artificial Sequence
  primer #59 (IL2_E61Q_F)
cttcagtgtctagaacaagaactcaaacctctg

SEQ ID NO: 273 - DNA, 33 bp, Artificial Sequence
  primer #60 (IL2_E61Q_R)
cagaggtttgagttcttgttctagacactgaag

SEQ ID NO: 274 - DNA, 30 bp, Artificial Sequence
  primer #61 (IL2_E61R_F)
cttcagtgtctagaacgggaactcaaacct

SEQ ID NO: 275 - DNA, 30 bp, Artificial Sequence
  primer #62 (IL2_E61R_R)
aggtttgagttcccgttctagacactgaag

SEQ ID NO: 276 - DNA, 33 bp, Artificial Sequence
  primer #63 (IL2_E68D_F)
ctcaaacctctggaggacgtgctaaatttagct

SEQ ID NO: 277 - DNA, 33 bp, Artificial Sequence
  primer #64 (IL2_E68D_R)
agctaaatttagcacgtcctccagaggtttgag

SEQ ID NO: 278 - DNA, 33 bp, Artificial Sequence
  primer #65 (IL2_E68Q_F)
ctcaaacctctggagcaggtgctaaatttagct

SEQ ID NO: 279 - DNA, 33 bp, Artificial Sequence
  primer #66 (IL2_E68Q_R)
agctaaatttagcacctgctccagaggtttgag

SEQ ID NO: 280 - DNA, 32 bp, Artificial Sequence
  primer #67 (IL2_V69G_F)
caaacctctggaggaagggctaaatttagctc

SEQ ID NO: 281 - DNA, 32 bp, Artificial Sequence
  primer #68 (IL2_V69G_R)
gagctaaatttagcccttcctccagaggtttg

SEQ ID NO: 282 - DNA, 40 bp, Artificial Sequence
  primer #69 (IL2_V69G_Q74A_F)
ctggaggaagggctaaatttagctgcaagcaaaaactttc

SEQ ID NO: 283 - DNA, 40 bp, Artificial Sequence
  primer #70 (IL2_V69G_Q74A_R)
gaaagtttttgcttgcagctaaatttagcccttcctccag

SEQ ID NO: 284 - DNA, 24 bp, Artificial Sequence
  primer #71 (IL2_Q74H_F)
ctaaatttagctcacagcaaaaac

SEQ ID NO: 285 - DNA, 24 bp, Artificial Sequence
  primer #72 (IL2_Q74H_R)
gtttttgctgtgagctaaatttag

SEQ ID NO: 286 - DNA, 33 bp, Artificial Sequence
  primer #73 (IL2_K76C_F)
aatttagctcaaagctgtaactttcacttaaga

SEQ ID NO: 287 - DNA, 33 bp, Artificial Sequence
  primer #74 (IL2_K76C_R)
tcttaagtgaaagttacagctttgagctaaatt

SEQ ID NO: 288 - DNA, 32 bp, Artificial Sequence
  primer #75 (IL2_L80D_R81E_F)
aaagcaaaaactttcacgacgaacccagggac

SEQ ID NO: 289 - DNA, 32 bp, Artificial Sequence
  primer #76 (IL2_L80D_R81E_R)
gtccctgggttcgtcgtgaaagtttttgcttt

SEQ ID NO: 290 - DNA, 29 bp, Artificial Sequence
  primer #77 (IL2_L80F_F)
gcaaaaactttcactttagacccagggac

SEQ ID NO: 291 - DNA, 29 bp, Artificial Sequence
  primer #78 (IL2_L80F_R)
gtccctgggtctaaagtgaaagtttttgc

SEQ ID NO: 292 - DNA, 29 bp, Artificial Sequence
  primer #79 (IL2_L80F_R81D_F)
gcaaaaactttcactttgaccccagggac

SEQ ID NO: 293 - DNA, 29 bp, Artificial Sequence
  primer #80 (IL2_L80F_R81D_R)
gtccctggggtcaaagtgaaagtttttgc

SEQ ID NO: 294 - DNA, 32 bp, Artificial Sequence
  primer #81 (IL2_L80F_R81E_F)
aaagcaaaaactttcacttcgaacccagggac

SEQ ID NO: 295 - DNA, 32 bp, Artificial Sequence
  primer #82 (IL2_L80F_R81E_R)
gtccctgggttcgaagtgaaagtttttgcttt

SEQ ID NO: 296 - DNA, 32 bp, Artificial Sequence
  primer #83 (IL2_L80V_R81D_F)
aaagcaaaaactttcacgtggatcccagggac

SEQ ID NO: 297 - DNA, 32 bp, Artificial Sequence
  primer #84 (IL2_L80V_R81D_R)
gtccctgggatccacgtgaaagtttttgcttt

SEQ ID NO: 298 - DNA, 32 bp, Artificial Sequence
  primer #85 (IL2_L80W_R81E_F)
aaagcaaaaactttcactgggaacccagggac

SEQ ID NO: 299 - DNA, 32 bp, Artificial Sequence
  primer #86 (IL2_L80W_R81E_R)
gtccctgggttcccagtgaaagtttttgcttt

SEQ ID NO: 300 - DNA, 29 bp, Artificial Sequence
  primer #87 (IL2_L80Y_R81D_F)
gcaaaaactttcactatgaccccagggac

SEQ ID NO: 301 - DNA, 29 bp, Artificial Sequence
  primer #88 (IL2_L80Y_R81D_R)
gtccctggggtcatagtgaaagtttttgc

SEQ ID NO: 302 - DNA, 32 bp, Artificial Sequence
  primer #89 (IL2_L80Y_R81E_F)
aaagcaaaaactttcactacgaacccagggac

SEQ ID NO: 303 - DNA, 32 bp, Artificial Sequence
  primer #90 (IL2_L80Y_R81E_R)
gtccctgggttcgtagtgaaagtttttgcttt

SEQ ID NO: 304 - DNA, 32 bp, Artificial Sequence
  primer #91 (IL2_L80Y_R81N_F)
aaagcaaaaactttcactacaaccccagggac

SEQ ID NO: 305 - DNA, 32 bp, Artificial Sequence
  primer #92 (IL2_L80Y_R81N_R)
gtccctggggttgtagtgaaagtttttgcttt

SEQ ID NO: 306 - DNA, 29 bp, Artificial Sequence
  primer #93 (IL2_L80Y_R81R_F)
gcaaaaactttcactatagacccagggac

SEQ ID NO: 307 - DNA, 29 bp, Artificial Sequence
  primer #94 (IL2_L80Y_R81R_R)
gtccctgggtctatagtgaaagtttttgc

SEQ ID NO: 308 - DNA, 31 bp, Artificial Sequence
  primer #95 (IL2_R81D_D84E_F)
ctttcacttagaccccagggagttaatcagc

SEQ ID NO: 309 - DNA, 31 bp, Artificial Sequence
  primer #96 (IL2_R81D_D84E_R)
gctgattaactccctggggtctaagtgaaag

SEQ ID NO: 310 - DNA, 34 bp, Artificial Sequence
  primer #97 (IL2_R81D_F)
caaaaactttcacttagaccccagggacttaatc

SEQ ID NO: 311 - DNA, 34 bp, Artificial Sequence
  primer #98 (IL2_R81D_R)
gattaagtccctggggtctaagtgaaagtttttg

SEQ ID NO: 312 - DNA, 51 bp, Artificial Sequence
  primer #99 (IL2_R81D_F_long)
ctcaaagcaaaaactttcacttagaccccagggacttaatcagcaaatatc

SEQ ID NO: 313 - DNA, 51 bp, Artificial Sequence
  primer #100 (IL2_R81D_R_long)
gatatttgctgattaagtccctggggtctaagtgaaagtttttgctttgag

SEQ ID NO: 314 - DNA, 43 bp, Artificial Sequence
  primer #101 (IL2_R81E_D84E_L85V_I86V_V91T_I92F_F)
gaacccagggaggtagtcagcaatatcaacacatttgttctgg

SEQ ID NO: 315 - DNA, 43 bp, Artificial Sequence
  primer #102 (IL2_R81E_D84E_L85V_I86V_V91T_I92F_R)
ccagaacaaatgtgttgatattgctgactacctccctgggttc

SEQ ID NO: 316 - DNA, 31 bp, Artificial Sequence
  primer #103 (IL2_R81E_F)
aaactttcacttagaacccagggacttaatc

SEQ ID NO: 317 - DNA, 31 bp, Artificial Sequence
  primer #104 (IL2_R81E_R)
gattaagtccctgggttctaagtgaaagttt

SEQ ID NO: 318 - DNA, 33 bp, Artificial Sequence
  primer #105 (IL2_P82G_F)
aactttcacttcgaaggcagggacgtagtcagc

SEQ ID NO: 319 - DNA, 33 bp, Artificial Sequence
  primer #106 (IL2_P82G_R)
gctgactacgtccctgccttcgaagtgaaagtt

SEQ ID NO: 320 - DNA, 33 bp, Artificial Sequence
  primer #107 (IL2_P82V_F)
aactttcacttcgaagtcagggacgtagtcagc

SEQ ID NO: 321 - DNA, 33 bp, Artificial Sequence
  primer #108 (IL2_P82V_R)
gctgactacgtccctgacttcgaagtgaaagtt

SEQ ID NO: 322 - DNA, 34 bp, Artificial Sequence
  primer #109 (IL2_D84E_F)
cttaagacccagggagttaatcagcaatatcaac

SEQ ID NO: 323 - DNA, 34 bp, Artificial Sequence
  primer #110 (IL2_D84E_R)
gttgatattgctgattaactccctgggtcttaag

SEQ ID NO: 324 - DNA, 32 bp, Artificial Sequence
  primer #111 (IL2_D84F_F)
cacttagaccccaggttcttaatcagcaatat

SEQ ID NO: 325 - DNA, 32 bp, Artificial Sequence
  primer #112 (IL2_D84F_R)
atattgctgattaagaacctggggtctaagtg

SEQ ID NO: 326 - DNA, 31 bp, Artificial Sequence
  primer #113 (IL2_D84V_F)
acttagaccccagggtcttaatcagcaatat

SEQ ID NO: 327 - DNA, 31 bp, Artificial Sequence
  primer #114 (IL2_D84V_R)
atattgctgattaagaccctggggtctaagt

SEQ ID NO: 328 - DNA, 35 bp, Artificial Sequence
  primer #115 (IL2_L85A_I86A_F)
ctttgaccccagggacgctgccagcaatatcaacg

SEQ ID NO: 329 - DNA, 35 bp, Artificial Sequence
  primer #116 (IL2_L85A_I86A_R)
cgttgatattgctggcagcgtccctggggtcaaag

SEQ ID NO: 330 - DNA, 30 bp, Artificial Sequence
  primer #117 (IL2_L85E_I86V_F)
cccagggacgaagtgagcaatatcaacgta

SEQ ID NO: 331 - DNA, 30 bp, Artificial Sequence
  primer #118 (IL2_L85E_I86V_R)
tacgttgatattgctcacttcgtccctggg

SEQ ID NO: 332 - DNA, 27 bp, Artificial Sequence
  primer #119 (IL2_L85F_I86L_F)
cccagggacttcctcagcaatatcaac

SEQ ID NO: 333 - DNA, 27 bp, Artificial Sequence
  primer #120 (IL2_L85F_I86L_R)
gttgatattgctgaggaagtccctggg

SEQ ID NO: 334 - DNA, 27 bp, Artificial Sequence
  primer #121 (IL2_L85F_I86V_F)
cccagggacttcgtcagcaatatcaac

SEQ ID NO: 335 - DNA, 27 bp, Artificial Sequence
  primer #122 (IL2_L85F_I86V_R)
gttgatattgctgacgaagtccctggg

SEQ ID NO: 336 - DNA, 27 bp, Artificial Sequence
  primer #123 (IL2_L85G_I86A_F)
cccagggacggagccagcaatatcaac

SEQ ID NO: 337 - DNA, 27 bp, Artificial Sequence
  primer #124 (IL2_L85G_I86A_R)
gttgatattgctggctccgtccctggg

SEQ ID NO: 338 - DNA, 35 bp, Artificial Sequence
  primer #125 (IL2_L85G_I86V_F)
ctttgaccccagggacggtgttagcaatatcaacg

SEQ ID NO: 339 - DNA, 35 bp, Artificial Sequence
  primer #126 (IL2_L85G_I86V_R)
cgttgatattgctaacccagtccctggggtcaaag

SEQ ID NO: 340 - DNA, 27 bp, Artificial Sequence
  primer #127 (IL2_L85I_I86V_F)
cccagggacatagtcagcaatatcaac

SEQ ID NO: 341 - DNA, 27 bp, Artificial Sequence
  primer #128 (IL2_L85I_I86V_R)
gttgatattgctgactatgtccctggg

SEQ ID NO: 342 - DNA, 34 bp, Artificial Sequence
  primer #129 (IL2_L85L_I86A_F)
cttcgaacccagggacctggccagcaatatcaac

SEQ ID NO: 343 - DNA, 34 bp, Artificial Sequence
  primer #130 (IL2_L85L_I86A_R)
gttgatattgctggccaggtccctgggttcgaag

SEQ ID NO: 344 - DNA, 34 bp, Artificial Sequence
  primer #131 (IL2_L85L_I86V_F)
ctttgagcccagggacttagtcagcaatatcaac

SEQ ID NO: 345 - DNA, 34 bp, Artificial Sequence
  primer #132 (IL2_L85L_I86V_R)
gttgatattgctgactaagtccctgggctcaaag

SEQ ID NO: 346 - DNA, 27 bp, Artificial Sequence
  primer #133 (IL2_L85T_I86G_F)
cccagggacacaggcagcaatatcaac

SEQ ID NO: 347 - DNA, 27 bp, Artificial Sequence
  primer #134 (IL2_L85T_I86G_R)
gttgatattgctgcctgtgtccctggg

SEQ ID NO: 348 - DNA, 29 bp, Artificial Sequence
  primer #135 (IL2_L85V_I86G_F)
cccagggacgtaggcagcaatatcaacgt

SEQ ID NO: 349 - DNA, 29 bp, Artificial Sequence
  primer #136 (IL2_L85V_I86G_R)
acgttgatattgctgcctacgtccctggg

SEQ ID NO: 350 - DNA, 31 bp, Artificial Sequence
  primer #137 (IL2_L85V_I86I_codon_F)
gaacccagggacgtaatcagcaatatcaacg

SEQ ID NO: 351 - DNA, 31 bp, Artificial Sequence
  primer #138 (IL2_L85V_I86I_codon_R)
cgttgatattgctgattacgtccctgggttc

SEQ ID NO: 352 - DNA, 30 bp, Artificial Sequence
  primer #139 (IL2_L85V_I86V_F)
gacccagggacgtagtcagcaatatcaacg

SEQ ID NO: 353 - DNA, 30 bp, Artificial Sequence
  primer #140 (IL2_L85V_I86V_R)
cgttgatattgctgactacgtccctgggtc

SEQ ID NO: 354 - DNA, 29 bp, Artificial Sequence
  primer #141 (IL2_L85W_I86V_F)
cccagggactgggtcagcaatatcaacgt

SEQ ID NO: 355 - DNA, 29 bp, Artificial Sequence
  primer #142 (IL2_L85W_I86V_R)
acgttgatattgctgacccagtccctggg

SEQ ID NO: 356 - DNA, 30 bp, Artificial Sequence
  primer #143 (IL2_L85W_I86V_Long_F)
tttgaccccagggactgggtcagcaatatc

SEQ ID NO: 357 - DNA, 30 bp, Artificial Sequence
  primer #144 (IL2_L85W_I86V_Long_R)
gatattgctgacccagtccctggggtcaaa

SEQ ID NO: 358 - DNA, 34 bp, Artificial Sequence
  primer #145 (IL2_L85Y_I86V_F)
cttcgaacccagggactacgtcagcaatatcaac

SEQ ID NO: 359 - DNA, 34 bp, Artificial Sequence
  primer #146 (IL2_L85Y_I86V_R)
gttgatattgctgacgtagtccctgggttcgaag

SEQ ID NO: 360 - DNA, 31 bp, Artificial Sequence
  primer #147 (IL2_I86V_V91T_I92F_F)
gtcagcaatatcaacacatttgttctggaac

SEQ ID NO: 361 - DNA, 31 bp, Artificial Sequence
  primer #148 (IL2_I86V_V91T_I92F_R)
gttccagaacaaatgtgttgatattgctgac

SEQ ID NO: 362 - DNA, 33 bp, Artificial Sequence
  primer #149 (IL2_S87C_F)
cccagggacttaatctgcaatatcaacgtaata

SEQ ID NO: 363 - DNA, 33 bp, Artificial Sequence
  primer #150 (IL2_S87C_R)
tattacgttgatattgcagattaagtccctggg

SEQ ID NO: 364 - DNA, 34 bp, Artificial Sequence
  primer #151 (IL2_N88F_F)
cagggacttaatcagctttatcaacgtatttgtt

SEQ ID NO: 365 - DNA, 34 bp, Artificial Sequence
  primer #152 (IL2_N88F_R)
aacaaatacgttgataaagctgattaagtccctg

SEQ ID NO: 366 - DNA, 33 bp, Artificial Sequence
  primer #153 (IL2_N88Q_F)
gggacttaatcagccaaatcaacgtaatagttc

SEQ ID NO: 367 - DNA, 33 bp, Artificial Sequence
  primer #154 (IL2_N88Q_R)
gaactattacgttgatttggctgattaagtccc

SEQ ID NO: 368 - DNA, 34 bp, Artificial Sequence
  primer #155 (IL2_N88V_F)
cagggacttaatcagcgttatcaacgtatttgtt

SEQ ID NO: 369 - DNA, 34 bp, Artificial Sequence
  primer #156 (IL2_N88V_R)
aacaaatacgttgataacgctgattaagtccctg

SEQ ID NO: 370 - DNA, 33 bp, Artificial Sequence
  primer #157 (IL2_I89F_F)
gacttaatcagcaatttcaacgtaatagttctg

SEQ ID NO: 371 - DNA, 33 bp, Artificial Sequence
  primer #158 (IL2_I89F_R)
cagaactattacgttgaaattgctgattaagtc

SEQ ID NO: 372 - DNA, 33 bp, Artificial Sequence
  primer #159 (IL2_V91E_I92F_F)
agcaatatcaacgaattcgttctggaactaaag

SEQ ID NO: 373 - DNA, 33 bp, Artificial Sequence
  primer #160 (IL2_V91E_I92F_R)
ctttagttccagaacgaattcgttgatattgct

SEQ ID NO: 374 - DNA, 33 bp, Artificial Sequence
  primer #161 (IL2_V91E_I92W_F)
agcaatatcaacgaatgggttctggaactaaag

SEQ ID NO: 375 - DNA, 33 bp, Artificial Sequence
  primer #162 (IL2_V91E_I92W_R)
ctttagttccagaacccattcgttgatattgct

SEQ ID NO: 376 - DNA, 34 bp, Artificial Sequence
  primer #163 (IL2_V91F_F)
cagcaatatcaactttatagttctggaactaaag

SEQ ID NO: 377 - DNA, 34 bp, Artificial Sequence
  primer #164 (IL2_V91F_R)
ctttagttccagaactataaagttgatattgctg

SEQ ID NO: 378 - DNA, 34 bp, Artificial Sequence
  primer #165 (IL2_V91T_F)
cagcaatatcaacacaatagttctggaactaaag

SEQ ID NO: 379 - DNA, 34 bp, Artificial Sequence
  primer #166 (IL2_V91T_R)
ctttagttccagaactattgtgttgatattgctg

SEQ ID NO: 380 - DNA, 32 bp, Artificial Sequence
  primer #167 (IL2_I92F_F)
gcaatatcaacgtatttgttctggaactaaag

SEQ ID NO: 381 - DNA, 32 bp, Artificial Sequence
  primer #168 (IL2_I92F_R)
ctttagttccagaacaaatacgttgatattgc

SEQ ID NO: 382 - DNA, 49 bp, Artificial Sequence
  primer #169 (IL2_I92F_F_long)
gacttaatcagcaatatcaacgtatttgttctggaactaaagggatctg

SEQ ID NO: 383 - DNA, 49 bp, Artificial Sequence
  primer #170 (IL2_I92F_R_long)
cagatccctttagttccagaacaaatacgttgatattgctgattaagtc

SEQ ID NO: 384 - DNA, 45 bp, Artificial Sequence
  primer #171 (IL2_I92F_F_long2)
cttaatcagcaatatcaacgtatttgttctggaactaaagggatc

SEQ ID NO: 385 - DNA, 45 bp, Artificial Sequence
  primer #172 (IL2_I92F_R_long2)
gatccctttagttccagaacaaatacgttgatattgctgattaag

SEQ ID NO: 386 - DNA, 32 bp, Artificial Sequence
  primer #173 (IL2_I92F_L94F_L96F_F)
caacgtatttgttttcgaattcaagggatctg

SEQ ID NO: 387 - DNA, 32 bp, Artificial Sequence
  primer #174 (IL2_I92F_L94F_L96F_R)
cagatcccttgaattcgaaaacaaatacgttg

SEQ ID NO: 388 - DNA, 39 bp, Artificial Sequence
  primer #175 (IL2_I92F_L94F_L96F_F)
gcaatatcaacgtatttgttttcgaatttaagggatctg

SEQ ID NO: 389 - DNA, 39 bp, Artificial Sequence
  primer #176 (IL2_I92F_L94F_L96F_R)
cagatcccttaaattcgaaaacaaatacgttgatattgc

SEQ ID NO: 390 - DNA, 39 bp, Artificial Sequence
  primer #177 (IL2_I92F_L94F_L96I_F)
gcaatatcaacgtatttgttttcgaaattaagggatctg

SEQ ID NO: 391 - DNA, 39 bp, Artificial Sequence
  primer #178 (IL2_I92F_L94F_L96I_R)
cagatcccttaatttcgaaaacaaatacgttgatattgc

SEQ ID NO: 392 - DNA, 39 bp, Artificial Sequence
  primer #179 (IL2_I92F_L94F_L96V_F)
gcaatatcaacgtatttgttttcgaagtaaagggatctg

SEQ ID NO: 393 - DNA, 39 bp, Artificial Sequence
  primer #180 (IL2_I92F_L94F_L96V_R)
cagatccctttacttcgaaaacaaatacgttgatattgc

SEQ ID NO: 394 - DNA, 33 bp, Artificial Sequence
  primer #181 (IL2_I92I_F)
gcaatatcaacgtaattgttctggaactaaagg

SEQ ID NO: 395 - DNA, 33 bp, Artificial Sequence
  primer #182 (IL2_I92I_R)
cctttagttccagaacaattacgttgatattgc

SEQ ID NO: 396 - DNA, 33 bp, Artificial Sequence
  primer #183 (IL2_I92L_F)
gcaatatcaacgtattagttctggaactaaagg

SEQ ID NO: 397 - DNA, 33 bp, Artificial Sequence
  primer #184 (IL2_I92L_R)
cctttagttccagaactaatacgttgatattgc

SEQ ID NO: 398 - DNA, 33 bp, Artificial Sequence
  primer #185 (IL2_I92W_F)
agcaatatcaacgtatgggttctggaactaaag

SEQ ID NO: 399 - DNA, 33 bp, Artificial Sequence
  primer #186 (IL2_I92W_R)
ctttagttccagaacccatacgttgatattgct

SEQ ID NO: 400 - DNA, 32 bp, Artificial Sequence
  primer #187 (IL2_I92Y_F)
gcaatatcaacgtatatgttctggaactaaag

SEQ ID NO: 401 - DNA, 32 bp, Artificial Sequence
  primer #188 (IL2_I92Y_R)
ctttagttccagaacatatacgttgatattgc

SEQ ID NO: 402 - DNA, 33 bp, Artificial Sequence
  primer #189 (IL2_L94F_L96F_F)
cgtaatagttttcgaatttaagggatctgaaac

SEQ ID NO: 403 - DNA, 33 bp, Artificial Sequence
  primer #190 (IL2_L94F_L96F_R)
gtttcagatcccttaaattcgaaaactattacg

SEQ ID NO: 404 - DNA, 33 bp, Artificial Sequence
  primer #191 (IL2_L94F_L96I_F)
cgtaatagttttcgaaattaagggatctgaaac

SEQ ID NO: 405 - DNA, 33 bp, Artificial Sequence
  primer #192 (IL2_L94F_L96I_R)
gtttcagatcccttaatttcgaaaactattacg

SEQ ID NO: 406 - DNA, 33 bp, Artificial Sequence
  primer #193 (IL2_L94F_L96V_F)
cgtaatagttttcgaagtaaagggatctgaaac

SEQ ID NO: 407 - DNA, 33 bp, Artificial Sequence
  primer #194 (IL2_L94F_L96V_R)
gtttcagatccctttacttcgaaaactattacg

SEQ ID NO: 408 - DNA, 30 bp, Artificial Sequence
  primer #195 (IL2_E95D_F)
gttctggacctaaagggatctgaaacaaca

SEQ ID NO: 409 - DNA, 30 bp, Artificial Sequence
  primer #196 (IL2_E95D_R)
tgttgtttcagatccctttaggtccagaac

SEQ ID NO: 410 - DNA, 33 bp, Artificial Sequence
  primer #197 (IL2_C125S_F)
agatggattacctttagtcaaagcatcatctca

SEQ ID NO: 411 - DNA, 33 bp, Artificial Sequence
  primer #198 (IL2_C125S_R)
tgagatgatgctttgactaaaggtaatccatct

SEQ ID NO: 412 - DNA, 34 bp, Artificial Sequence
  primer #199 (IL2_Q126T_F)
gatggattacctttagtacaagcatcatctcaac

SEQ ID NO: 413 - DNA, 34 bp, Artificial Sequence
  primer #200 (IL2_Q126T_R)
gttgagatgatgcttgtactaaaggtaatccatc

SEQ ID NO: 414 - DNA, 33 bp, Artificial Sequence
  primer #201 (IL2_desA1_F)
taagaatatacatatgcctacttcaagttctac

SEQ ID NO: 415 - DNA, 33 bp, Artificial Sequence
  primer #202 (IL2_desA1_R)
gtagaacttgaagtaggcatatgtatattctta

SEQ ID NO: 416 - DNA, 34 bp, Artificial Sequence
  primer #203 (IL2_NdeI_desA1_N-term)
cgccatatgcctacttcaagttctacaaagaaaa

SEQ ID NO: 417 - DNA, 34 bp, Artificial Sequence
  primer #204 (IL2_BHI_C-term)
cgggatcctcaagtcagtgttgagatgatgcttt

SEQ ID NO: 418 - protein, 12 aa, HOMO SAPIENS
ESKYGPPCPSCP

SEQ ID NO: 419 - protein, 11 aa, Artificial Sequence
  Variant of hinge region
ESKYGPPPSCP

SEQ ID NO: 420 - protein, 11 aa, Artificial Sequence
  Variant of hinge region
ESKYGPPCPSP

SEQ ID NO: 421 - protein, 10 aa, Artificial Sequence
  Variant of hinge region
ESKYGPPCPS

SEQ ID NO: 422 - protein, 10 aa, Artificial Sequence
  Variant of hinge region
ESKYGPPCPP

SEQ ID NO: 423 - protein, 8 aa, Artificial Sequence
  Variant of hinge region
KYGPPCPS

SEQ ID NO: 424 - protein, 8 aa, Artificial Sequence
  Variant of hinge region
ESKYGPPC

SEQ ID NO: 425 - protein, 7 aa, Artificial Sequence
  Variant of hinge region
EKYGPPC

SEQ ID NO: 426 - protein, 6 aa, Artificial Sequence
  Variant of hinge region
ESPSCP

SEQ ID NO: 427 - protein, 5 aa, Artificial Sequence
  Variant of hinge region
EPSCP

SEQ ID NO: 428 - protein, 4 aa, Artificial Sequence
  Variant of hinge region
PSCP

SEQ ID NO: 429 - protein, 10 aa, Artificial Sequence
  Variant of hinge region
ESKYGPPSCP

SEQ ID NO: 430 - protein, 9 aa, Artificial Sequence
  Variant of hinge region
KYGPPPSCP

SEQ ID NO: 431 - protein, 9 aa, Artificial Sequence
  Variant of hinge region
ESKYGPSCP

SEQ ID NO: 432 - protein, 8 aa, Artificial Sequence
  Variant of hinge region
ESKYGPPC

SEQ ID NO: 433 - protein, 7 aa, Artificial Sequence
  Variant of hinge region
KYGPPCP

SEQ ID NO: 434 - protein, 7 aa, Artificial Sequence
  Variant of hinge region
ESKPSCP

SEQ ID NO: 435 - protein, 6 aa, Artificial Sequence
  Variant of hinge region
ESPSCP

SEQ ID NO: 436 - protein, 4 aa, Artificial Sequence
  Variant of hinge region
EPSC

SEQ ID NO: 437 - protein, 3 aa, Artificial Sequence
  Variant of hinge region
SCP

SEQ ID NO: 438 - protein, 221 aa, homo sapiens
PSCPAPEFLGGPSVFLFPPKPKDTLMISRTPEVTCVVVDVSQEDPEVQFNWYVDGVEVHNAKTKPREEQFNSTYRVVSVLTVLHQDWLNGKEYKCKVSNKGLPSSIEKTISKAKGQPREPQVYTLPPSQEEMTKNQVSLTCLVKGFYPSDIAVEWESNGQPENNYKTTPPVLDSDGSFFLYSRLTVDKSRWQEGNVFSCSVMHEALHNHYTQKSLSLSLGK

SEQ ID NO: 439 - protein, 442 aa, Homo sapiens
  MISC_FEATURE (1)..(442): Amino acids at position 1 to 442 form Human Immunoglobulin G4 Fc Fragment (homodimer)
  MISC_FEATURE (1)..(221): Amino acids at position 1 to 221 form one monomer
  MISC_FEATURE (222)..(442): Amino acids at position 222 to 442 form one monomer
  DISULFID (3)..(224): Amino acids at position 3 and position 224 form an inter-disulfide bond
  DISULFID (35)..(95): Amino acids at position 35 and position 95 form an intra-chain disulfide bond
  DISULFID (141)..(199): Amino acids at position 141 and position 199 form an intra-chain disulfide bond
  DISULFID (256)..(316): Amino acids at position 256 and position 316 form an intra-chain disulfide bond
  DISULFID (362)..(420): Amino acids at position 362 and position 420 form an intra-chain disulfide bond
PSCPAPEFLGGPSVFLFPPKPKDTLMISRTPEVTCVVVDVSQEDPEVQFNWYVDGVEVHNAKTKPREEQFNSTYRVVSVLTVLHQDWLNGKEYKCKVSNKGLPSSIEKTISKAKGQPREPQVYTLPPSQEEMTKNQVSLTCLVKGFYPSDIAVEWESNGQPENNYKTTPPVLDSDGSFFLYSRLTVDKSRWQEGNVFSCSVMHEALHNHYTQKSLSLSLGKPSCPAPEFLGGPSVFLFPPKPKDTLMISRTPEVTCVVVDVSQEDPEVQFNWYVDGVEVHNAKTKPREEQFNSTYRVVSVLTVLHQDWLNGKEYKCKVSNKGLPSSIEKTISKAKGQPREPQVYTLPPSQEEMTKNQVSLTCLVKGFYPSDIAVEWESNGQPENNYKTTPPVLDSDGSFFLYSRLTVDKSRWQEGNVFSCSVMHEALHNHYTQKSLSLSLGK